European Patent Application EP 4 248 976 A2, published September 27, 2023. Title: ANTIGEN BINDING PROTEINS TO PROPROTEIN CONVERTASE SUBTILISIN KEXIN TYPE 9 (PCSK9). Applicant: AMGEN INC. The sequence listing filed with the application follows.

SEQUENCE LISTING (499 sequences)

SEQ ID NO: 1 - protein, 662 aa, Homo sapiens
QEDEDGDYEELVLALRSEEDGLAEAPEHGTTATFHRCAKDPWRLPGTYVVVLKEETHLSQSERTARRLQAQAARRGYLTKILHVFHGLLPGFLVKMSGDLLELALKLPHVDYIEEDSSVFAQSIPWNLERITPPRYRADEYQPPDGGSLVEVYLLDTSIQSDHREIEGRVMVTDFENVPEEDGTRFHRQASKCDSHGTHLAGVVSGRDAGVAKGASMRSLRVLNCQGKGTVSGTLIGLEFIRKSQLVQPVGPLVVLLPLAGGYSRVLNAACQRLARAGVVLVTAAGNFRDDACLYSPASAPEVITVGATNAQDQPVTLGTLGTNFGRCVDLFAPGEDIIGASSDCSTCFVSQSGTSQAAAHVAGIAAMMLSAEPELTLAELRQRLIHFSAKDVINEAWFPEDQRVLTPNLVAALPPSTHGAGWQLFCRTVWSAHSGPTRMATAIARCAPDEELLSCSSFSRSGKRRGERMEAQGGKLVCRAHNAFGGEGVYAIARCCLLPQANCSVHTAPPAEASMGTRVHCHQQGHVLTGCSSHWEVEDLGTHKPPVLRPRGQPNQCVGHREASIHASCCHAPGLECKVKEHGIPAPQGQVTVACEEGWTLTGCSALPGTSHVLGAYAVDNTCVVRSRDVSTTGSTSEEAVTAVAICCRSRHLAQASQELQ

SEQ ID NO: 2 - DNA, 2076 bp, Homo sapiens
  source 1..2076: mol_type = unassigned DNA
atgggcaccgtcagctccaggcggtcctggtggccgctgccactgctgctgctgctgctgctgctcctgggtcccgcgggcgcccgtgcgcaggaggacgaggacggcgactacgaggagctggtgctagccttgcgctccgaggaggacggcctggccgaagcacccgagcacggaaccacagccaccttccaccgctgcgccaaggatccgtggaggttgcctggcacctacgtggtggtgctgaaggaggagacccacctctcgcagtcagagcgcactgcccgccgcctgcaggcccaggctgcccgccggggatacctcaccaagatcctgcatgtcttccatggccttcttcctggcttcctggtgaagatgagtggcgacctgctggagctggccttgaagttgccccatgtcgactacatcgaggaggactcctctgtctttgcccagagcatcccgtggaacctggagcggattacccctccgcggtaccgggcggatgaataccagccccccgacggaggcagcctggtggaggtgtatctcctagacaccagcatacagagtgaccaccgggaaatcgagggcagggtcatggtcaccgacttcgagaatgtgcccgaggaggacgggacccgcttccacagacaggccagcaagtgtgacagtcatggcacccacctggcaggggtggtcagcggccgggatgccggcgtggccaagggtgccagcatgcgcagcctgcgcgtgctcaactgccaagggaagggcacggttagcggcaccctcataggcctggagtttattcggaaaagccagctggtccagcctgtggggccactggtggtgctgctgcccctggcgggtgggtacagccgcgtcctcaacgccgcctgccagcgcctggcgagggctggggtcgtgctggtcaccgctgccggcaacttccgggacgatgcctgcctctactccccagcctcagctcccgaggtcatcacagttggggccaccaatgcccaggaccagccggtgaccctggggactttggggaccaactttggccgctgtgtggacctctttgccccaggggaggacatcattggtgcctccagcgactgcagcacctgctttgtgtcacagagtgggacatcacaggctgctgcccacgtggctggcattgcagccatgatgctgtctgccgagccggagctcaccctggccgagttgaggcagagactgatccacttctctgccaaagatgtcatcaatgaggcctggttccctgaggaccagcgggtactgacccccaacctggtggccgccctgccccccagcacccatggggcaggttggcagctgttttgcaggactgtgtggtcagcacactcggggcctacacggatggccacagccatcgcccgctgcgccccagatgaggagctgctgagctgctccagtttctccaggagtgggaagcggcggggcgagcgcatggaggcccaagggggcaagctggtctgccgggcccacaacgcttttgggggtgagggtgtctacgccattgccaggtgctgcctgctaccccaggccaactgcagcgtccacacagctccaccagctgaggccagcatggggacccgtgtccactgccaccaacagggccacgtcctcacaggctgcagctcccactgggaggtggaggaccttggcacccacaagccgcctgtgctgaggccacgaggtcagcccaaccagtgcgtgggccacagggaggccagcatccacgcttcctgctgccatgccccaggtctggaatgcaaagtcaaggagcatggaatcccggcccctcaggggcaggtgaccgtggcctgcgaggagggctggaccctgactggctgcagcgccctccctgggacctcccacgtcctgggggcctacgccgtagacaacacgtgtgtagtcaggagccgggacgtcagcactacaggcagcaccagcgaagaggccgtgacagccgttgccatctgctgccggagccggcacctggcgcaggcctcccaggagctccag

SEQ ID NO: 3 - protein, 692 aa, Homo sapiens
MGTVSSRRSWWPLPLLLLLLLLLGPAGARAQEDEDGDYEELVLALRSEEDGLAEAPEHGTTATFHRCAKDPWRLPGTYVVVLKEETHLSQSERTARRLQAQAARRGYLTKILHVFHGLLPGFLVKMSGDLLELALKLPHVDYIEEDSSVFAQSIPWNLERITPPRYRADEYQPPDGGSLVEVYLLDTSIQSDHREIEGRVMVTDFENVPEEDGTRFHRQASKCDSHGTHLAGVVSGRDAGVAKGASMRSLRVLNCQGKGTVSGTLIGLEFIRKSQLVQPVGPLVVLLPLAGGYSRVLNAACQRLARAGVVLVTAAGNFRDDACLYSPASAPEVITVGATNAQDQPVTLGTLGTNFGRCVDLFAPGEDIIGASSDCSTCFVSQSGTSQAAAHVAGIAAMMLSAEPELTLAELRQRLIHFSAKDVINEAWFPEDQRVLTPNLVAALPPSTHGAGWQLFCRTVWSAHSGPTRMATAIARCAPDEELLSCSSFSRSGKRRGERMEAQGGKLVCRAHNAFGGEGVYAIARCCLLPQANCSVHTAPPAEASMGTRVHCHQQGHVLTGCSSHWEVEDLGTHKPPVLRPRGQPNQCVGHREASIHASCCHAPGLECKVKEHGIPAPQGQVTVACEEGWTLTGCSALPGTSHVLGAYAVDNTCVVRSRDVSTTGSTSEEAVTAVAICCRSRHLAQASQELQ

SEQ ID NO: 4 - protein, 112 aa, Homo sapiens
DIVMTQSPLSLPVTPGEPASISCRSSQSLLHSNGYNYLDWYLQKPGQSPQLLIYLGSNRASGVPDRFSGSGSGTDFTLKISRVEAEDVGVYYCMQALQTPFTFGPGTKVDIK

SEQ ID NO: 5 - protein, 112 aa, Homo sapiens
DIVMTQSPLSLSVTPGEPPSISCRSSQSLLHSNGYNFLNWYLQKPGQSPQLLIYLGSHRASGVPDRFSGSGSGTDFTLEISRVEAEDVGVYYCMQVLQTPFTFGPGTKVDIK

SEQ ID NO: 6 - protein, 107 aa, Homo sapiens [sequence omitted]

SEQ ID NO: 7 - protein, 107 aa, Homo sapiens
DIQMTQSPSSLSASVGDRVTITCRASQRISNYLSWYLQKPGIAPKLLIYAASSLQSGVPSRFSGSGSGTDFTLTISSLQSEDFATYYCQQSYSTPLIFGGGTKVEIK

SEQ ID NO: 8 - protein, 107 aa, Homo sapiens
DIQMTQSPSSLSASVGDRVTITCRASQSISSYLNWYQQKPGKAPKLLIYAASSLQSGVPSRFSGSGSGTDFTLTISSLQPEDFATYYCQQSYSTPITFGQGTRLEIK

SEQ ID NO: 9 - protein, 107 aa, Homo sapiens
DILMTQSPSSLSASVGDRVTITCRASQSISSYLNWYQQKPGKAPKVLIYAASSLQSGVPSRFSGSGSGTDFTLTINSLQPEDFATYYCQQSYSSPITFGQGTRLEIK

SEQ ID NO: 10 - protein, 107 aa, Homo sapiens
DIQMTQSPSSLSASVGDRVTITCRASQSISIYLNWYQQKPGKAPYLLIYAAASLQSGVPSRFSGSGSGTDFTLTISSLQPEDFATYYCQQSYSAPITFGQGTRLEIK

SEQ ID NO: 11 - protein, 111 aa, Homo sapiens
QSVLTQPPSVSGAPGQRVTISCTGSSSNIGAGYDVHWYQQLPGTAPKLLIYGNSNRPSGVPDRFSGSKSGTSASLAITGLQAEDEADYYCQSYDSSLSGSVFGGGTKLTVL

SEQ ID NO: 12 - protein, 111 aa, Homo sapiens
QSVLTQPPSVSGAPGQRVTISCTGSSSNIGAGYDVHWYQQLPGTAPKLLISGNSNRPSGVPDRFSGSKSGTSASLAITGLQAEDEADYYCQSYDSSLSGSVFGGGTKLTVL

SEQ ID NO: 13 - protein, 111 aa, Homo sapiens
QSVLTQPPSVSGAPGQRVTISCTGSSSNIGAHYDVHWYQQVPGTAPKLLIYGNTYRPSGVPDRFSGSKSGTSASLAITGLQAEDEADYYCQSYDNSLSGVVFGGGTKLTVL

SEQ ID NO: 14 - protein, 108 aa, Homo sapiens
QSALTQPASVSGSPGQSITISCTGTSSDVGGYNYVSWYQQHPGKAPKLMIYEVSNRPSGVSNRFSGSKSGNTASLTISGLQAEDEADYYCSSYTSSSVFGGGTKLTVL

SEQ ID NO: 15 - protein, 109 aa, Homo sapiens
QSALTQPASVSGSPGQSITISCTGTSSDVGRYNSVSWYQHHPGKAPKVMIYEVSNRPSGVSTRFSGSKSGNTASLTISGLQAEDEADYYCSSYTSSSVVFGGGTKLTVL

SEQ ID NO: 16 - protein, 109 aa, Homo sapiens
QSALTQPASVSGSPGQSITISCTGTSSDVGGYNSVSWYQQHPGKPPKLMIYEVSNRPSGVSIRFSGSKSGNTASLTISGLQAEDEADYFCSSYTSTSMVFGGGTKLTVL

SEQ ID NO: 17 - protein, 109 aa, Homo sapiens; identical to SEQ ID NO: 16

SEQ ID NO: 18 - protein, 109 aa, Homo sapiens
QSALTQPASVSGSPGQSITISCTGTSSDVGGYNSVSWYQQHPGKPPKLMIYEVSNRPSGVSNRFSGSKSGNTASLTISGLQAEDEADYFCSSYTSTSMVFGGGTKLAVL

SEQ ID NO: 19 - protein, 109 aa, Homo sapiens
QSALTQPASVSGSPGQSITISCTGTSSDVGGYNSVSWYQQYPGKPPKLKIYEVSNRPSGVSNRFSGSKSGNTASLTISGLQAEDEADYFCSSYTSTSMVFGGGTKLTVL

SEQ ID NO: 20 - protein, 109 aa, Homo sapiens
QSALTQPASVSGSPGQSITISCTGTSSDVGGYNSVSWYQQHPGKPPKLMIYEVSNRPSGVSNRFSGSKSGNTASLTISGLQAEDEADYFCSSYTSTSMVFGGGTKLTVL

SEQ ID NO: 21 - protein, 109 aa, Homo sapiens; identical to SEQ ID NO: 20

SEQ ID NO: 22 - protein, 109 aa, Homo sapiens
QSALTQPASVSGSPGQSITISCTGTNSDVGGYNSVSWYQQHPGKPPKLMIYEVSNRPSGISNRFSGSKSGNTASLTISGLQAEDEADYFCSSYTSTSMVFGGGTKLTVL

SEQ ID NO: 23 - protein, 109 aa, Homo sapiens
QSALTQPASVSGSPGQSITISCTGTSSDVGGYNSVSWYQQHPGKAPKLMIYEVSNRPSGVSNRFSGSKSGNTASLTISGLQAEDEADYYCNSYTSTSMVFGGGTKLTVL

SEQ ID NO: 24 - protein, 109 aa, Homo sapiens
QSALTQPASVSGSPGQSITISCTGTSSDVGAYNSVSWYQQHPGKAPKRMIYEVSNRPSGVSNRFSGSKSGNTASLTISGLQAEDEADYYCSSYTSTNMVFGGGTKLTVL

SEQ ID NO: 25 - protein, 108 aa, Homo sapiens; identical to SEQ ID NO: 14

SEQ ID NO: 26 - protein, 109 aa, Homo sapiens
QSALTQPASVSGSPGQSITISCTGTSSDVGGYNSVSWYQQHPGKAPKLMIYEVTNRPSGVSNRFSGSKSGNTASLTISGLQAEDEADYYCNSYTSTSMVFGGGTKLTVL

SEQ ID NO: 27 - protein, 108 aa, Homo sapiens
QSALTQPASVSGSPGQSITISCTGTSSDVGSYNLVSWYQQHPGKAPKLMIYEGSKRPSGVSNRFSGSKSGNTASLTISGLQAEDEADYYCCSYAGSSTFGGGTKLTVL

SEQ ID NO: 28 - protein, 110 aa, Homo sapiens
LSALTQPASVSGSPGQSITISCTGTSSDVGNYNLVSWYQQYSGKAPKLMIYEVSKRPSGVSNRFSGSKSGNTASLTISGLQAEDEADYYCCSYAGSSTLVFGGGTKLTVL

SEQ ID NO: 29 - protein, 108 aa, Homo sapiens
QSVLTQPPSASGTPGQRVTISCSGSSSNIGSNTVNWYQQLPGTAPKLLIYSNNQRPSGVPDRFSGSKSGTSASLAISGLQSEDEADYYCAAWDDSLNVFGGGTKLTVL

SEQ ID NO: 30 - protein, 109 aa, Homo sapiens
QSVLTQPPSASGTPGQRVTISCSGSSSNIGSKTVNWYQQVPGTAPKLLIYRNNQRPLGVPDRFSGSKSGTSASLAISGLQSEDEADYYCAAWDDSLNWVFGGGTKLTVL

SEQ ID NO: 31 - protein, 109 aa, Homo sapiens
QSVLTQPPSASGPPGQRVTISCSGSSSNIGSNTVNWYQQLPGTAPKLLIYSNNRRPSGVPDRFSGSKSGTSASLAISGLQSEDEADYYCAAWDDSLNWVFGGGTKLTVL

SEQ ID NO: 32 - protein, 110 aa, Homo sapiens
QSVLTQPPSASGTPGQRVTISCSGSSSNIGSNTVNWYQQLPGTAPKLLIYSNNQRPSGVPDRFSGSKSGTSASLAISGLQSEDEADYYCAVWDDSLNGWVFGGGTKLTVL

SEQ ID NO: 33 - protein, 109 aa, Homo sapiens
QSVLTQPPSASGTPGQRVTISCSGSSSNIGSKTVNWYQQFPGTAPKLLIYSNNRRPSGVPDRFSGSKSGTSASLAISGLQSEDEADYYCAAWDDSLNWVFGAGTKLTVL

SEQ ID NO: 34 - protein, 110 aa, Homo sapiens
QSVLTQPPSVSAAPGQKVTISCSGSSSNIGNNYVSWYQQLPGTAPKLLIYDNNKRPSGIPDRFSGSKSGTSATLGITGLQTGDEADYYCGTWDSSLSAYVFGTGTKVTVL

SEQ ID NO: 35 - protein, 110 aa, Homo sapiens
QSVLTQPPSVSAAPGQKVTISCSGSSSNIGNNFVSWYQQLPGTAPKLLIYDYNKRPSGIPDRFSGSKSGTSATLGITGLQTGDEADYYCGTWDSSLSAYVFGTGTRVTVL

SEQ ID NO: 36 - protein, 110 aa, Homo sapiens
QSVLTQPPSVSAAPGQKVTISCSGSSSNIGNNFVSWYQQLPGTAPKLLIYDYNKRPSGIPDRFSGSKSGTSATLGITGLQTGDEADYYCGTWDSSLSGYVFGTGTRVTVL

SEQ ID NO: 37 - protein, 110 aa, Homo sapiens
QSVLTQPPSVSAAPGQKVTISCSGSSSNIGNNFVSWYQQFPGTAPKLLIYDYNKRPSGIPDRFSGSKSGTSATLGITGLQTGDEADYYCGTWDSSLSSYVFGTGTRVTVL

SEQ ID NO: 38 - protein, 110 aa, Homo sapiens; identical to SEQ ID NO: 36

SEQ ID NO: 39 - protein, 110 aa, Homo sapiens
QSVLTQPPTVSAAPGQKVTISCSGSSSNIGNNFVSWYQQLPGTAPKLLIYDYNKRPSGIPDRFSGSKSGTSATLGITGLQTGDEADYYCGTWDSSLSGYVFGTGTRVTVL

SEQ ID NO: 40 - protein, 110 aa, Homo sapiens
QSVLTQPPSVSAAPGQKVTISCSGSSSNIGNNFVSWYQQLPGTAPKLLIYDSNKRPSGIPDRFSGSKSGTSATLDITGLQTGDEADYYCGTWDSSLSAYVFGTGTKVTVL

SEQ ID NO: 41 - protein, 110 aa, Homo sapiens
QSVLTQPPSVSAAPGQKVTISCSGSSSNIGNNYVSWYQQLPGTAPKLLIYDNNKRPSGIPDRFSGSKSGTSATLGITGLQTGDEADYYCGTWDSSLSAVVFGGGTKLTVL

SEQ ID NO: 42 - protein, 110 aa, Homo sapiens
QSVLTQPPSVSAAPGQKVTISCSGSNSNIGNNYVSWYQQLPGTAPKLLIYDNNKRPSGIPDRFSGSNSGTSATLGITGLQTGDEADYYCGTWDSSLSAVVFGGGTKLTVL

SEQ ID NO: 43 - protein, 107 aa, Homo sapiens
SYELTQPPSVSVSPGQTASITCSGDKLGDKYACWYQQKPGQSPVLVIYQDSKRPSGIPERFSGSNSGNTATLTISGTQAMDEADYYCQAWDSSTAVVFGGGTKLTVL

SEQ ID NO: 44 - protein, 106 aa, Homo sapiens
SYELTQPPSVSVSPGQTARITCSGDKLGDKYACWYQQKPGQSPVLVIYQNTKWPLGIPERFSGSKSGNTVTLTISGTQAMDEADYYCQAWDSSTVVFGGGTKLTVL

SEQ ID NO: 45 - protein, 116 aa, Homo sapiens
QPVLTQPPSASASLGASVTLTCTLSSGYSNYKVDWYQQRPGKGPRFVMRVGTGGIVGSKGDGIPDRFSVLGSGLNRYLTIKNIQEEDESDYHCGADHGSGSNFVVVFGGGTKLTVL

SEQ ID NO: 46 - protein, 116 aa, Homo sapiens
QPVLTQPLFASASLGASVTLTCTLSSGYSSYEVDWYQQRPGKGPRFVMRVDTGGIVGSKGEGIPDRFSVLGSGLNRYLTIKNIQEEDESDYHCGADHGSGTNFVVVFGGGTKLTVL

SEQ ID NO: 47 - protein, 114 aa, Homo sapiens
QVQLVQSGAEVKKPGASVKVSCKASGYTFTSYGISWVRQAPGQGLEWMGWISAYNGNTNYAQKLQGRVTMTTDTSTSTAYMELRSLRSDDTAVYYCARYGMDVWGQGTTVTVSS

SEQ ID NO: 48 - protein, 115 aa, Homo sapiens
QIQLVQSGAEVKKPGASVKVSCKASGYPLTSYGISWVRQAPGQGLEWMGWISAYNGNTNYAQKVQGSVTMTTDTSTSTVYMELRSLRSDDTAVYYCARGYGMDVWGQGTTVTVSS

SEQ ID NO: 49 - protein, 115 aa, Homo sapiens
QVQLVQSGAEVKKPGASVKVSCKASGYTLTSYGISWVRQAPGQGLEWMGWVSFYNGNTNYAQKLQGRGTMTTDPSTSTAYMELRSLRSDDTAVYYCARGYGMDVWGQGTTVTVSS

SEQ ID NO: 50 - protein, 115 aa, Homo sapiens; identical to SEQ ID NO: 49

SEQ ID NO: 51 - protein, 115 aa, Homo sapiens
QVQLVQSGAEVKKPGASVKVSCKASGYTLTSYGISWVRQAPGQGLEWMGWISFYNGNTNYAQKVQGRVTMTTDTSTSTVYMELRSLRSDDTAVYYCARGYGMDVWGQGTTVTVSS

SEQ ID NO: 52 - protein, 115 aa, Homo sapiens
QVQLVQSGAEVKRPGASVKVSCKASGYTLTSYGISWVRQAPGQGLEWMGWISVYNGNTNYAQKVQGRVTMTTDTSTSTVYMELRSLSSDDTAVYYCARGYGMDVWGQGTTVTVSS

SEQ ID NO: 53 - protein, 115 aa, Homo sapiens
QIQLVQSGAEVKKPGASVKVSCKASGYTLTSYGISWVRQAPGQGLEWMGWISFYNGNTNYAQKVQGRVTMTTDTSTSTVYMELRSLRSDDTAVYFCARGYGMDVWGQGTTVTVSS

SEQ ID NO: 54 - protein, 115 aa, Homo sapiens
QVQLVQSGAEVKKPGASLKVSCKASGYSLTSYGISWVRQAPGQGLEWMGWISAYNGNTNYAQKVQGRVTMTTDTSTSTVYMEVRSLRSDDTAVYYCARGYGMDVWGQGTTVTVSS

SEQ ID NO: 55 - protein, 115 aa, Homo sapiens
QVQLVQSGAEVKKPGASVKVSCKASGYPLTSYGISWVRQAPGQGLEWMGWISAYNGNTNYAQKVQGRVTMTTDTSTSTVYMELRSLRSDDTAVYYCARGYGMDVWGQGTTVTVSS

SEQ ID NO: 56 - protein, 115 aa, Homo sapiens
QVQLVQSGAEVKKPGASVKVSCKASGYALTSYGISWVRQAPGQGLEWMGWISAYNGNTNYAQKVQGRVTMTTDTSTSTVYMELRSLRSDDTAVYYCARGYGMDVWGQGTTVTVSS

SEQ ID NO: 57 - protein, 115 aa, Homo sapiens
QVQLVQSGAEVKKPGASVKVSCKASGYSFTSYGISWVRQAPGQGLEWMGWVSAYNGNTNYAQKFQGRVTMTTDTSTSTAYMELRSLRSDDTAVYYCARGYVMDVWGQGTTVTVSS

SEQ ID NO: 58 - protein, 115 aa, Homo sapiens
QVQLVQSGAEVKKPGASVKVSCKASGYTFPSYGISWVRQAPGQGLEWMGWISAYNGNTNYAEKLQGRVTMTTDTSTSTAYMEVRSLRSDDTAVFYCARGYVMDVWGQGTTVTVSS

SEQ ID NO: 59 - protein, 113 aa, Homo sapiens
QVQLVQSGAEVKKPGASVKVSCKASGYTFTSYGISWVRQAPGQGLEWMGWISAYNGNTNYAQKLQGRVTMTTDTSTSTAYMELRSLRSDDTAVYYCARGYDYWGQGTLVTVSS

SEQ ID NO: 60 - protein, 115 aa, Homo sapiens
QVQLVQSGAEVKKPGASVKVSCKASGYTFTSYGISWVRQAPGQGLEWMGWISTYNGNTNYAQKVQGRVTMTTDTSTSTAYMELRSLRSDDTAVYYCARGYTRDYWGQGTLVTVSS

SEQ ID NO: 61 - protein, 116 aa, Homo sapiens
EVQLVESGGGLVQPGGSLRLSCAASGFTFSSYWMSWVRQAPGKGLEWVANIKQDGSEKYYVDSVKGRFTISRDNAKNSLYLQMNSLRAEDTAVYYCARNWGAFDVWGQGTMVTVSS

SEQ ID NO: 62 - protein, 119 aa, Homo sapiens
EVQLVESGGGLVQPGGSLRLSCAASGFTFSRYWMSWVRQAPGKGLEWVANIKHDGSEKYYVDSVKGRFTISRDNAKNSLYLQMNSLRAEDTAVYYCARESNWGFAFDVWGHGTMVTVSS

SEQ ID NO: 63 - protein, 116 aa, Homo sapiens
EVQLVESGGGLVQPGGSLRLSCAASGFTFSSYWMSWVRQAPGKGLEWVANIKQDGSEKYYVDSVKGRFTISRDNAKNSLYLQMNSLRAEDTAVYYCARNWGAFDIWGQGTMVTVSS

SEQ ID NO: 64 - protein, 119 aa, Homo sapiens
EVQLVESGGGLVQPGGSLRLSCVVSGFTFSSYWMSWVRQAPGKGLEWVANIKQDGSEKYYVDSVKGRFTISRDNAKNSLYLQMNSLRAEDTAVYYCARESNWGFAFDIWGQGTMVTVSS

SEQ ID NO: 65 - protein, 119 aa, Homo sapiens
EVQLVESGGGLVQPGGSLRLSCAASGLTFSNFWMSWVRQAPGKGLEWVANIKQDGSEKYYVDSVKGRFTISRDNAKNSLYLQMNSLRAEDTAVYSCTRESNWGFAFDIWGQGTMVTVSS

SEQ ID NO: 66 - protein, 123 aa, Homo sapiens
EVQLVESGGGLVKPGGSLRLSCAASGFTFSSYSMNWVRQAPGKGLEWVSSISSSSSYIYYADSVKGRFTISRDNAKNSLYLQMNSLRAEDTAVYYCARDYDFWSGYYTAFDVWGQGTMVTVSS

SEQ ID NO: 67 - protein, 123 aa, Homo sapiens
EVQLVESGGGLVKPGGSLRLSCAASGFTFSSYSMNWVRQAPGKGLEWVSSISSSSSYISYADSVKGRFTISRDNAKNSLYLQMNSLRAEDTAVYFCARDYDFWSAYYDAFDVWGQGTMVTVSS

SEQ ID NO: 68 - protein, 112 aa, Homo sapiens
EVQLLESGGGLVQPGGSLRLSCAASGFTFSSYAMSWVRQAPGKGLEWVSAISGSGGSTYYADSVKGRFTISRDNSKNTLYLQMNSLRAEDTAVYYCAKFDYWGQGTLVTVSS

SEQ ID NO: 69 - protein, 117 aa, Homo sapiens
EVQLLESGGGLVQPGGSLRLSCAASGFTFSSYAMSWVRQAPGKGLEWVSTISGSGGRTYYADSVKGRFTISRDNSKNTLYLQMNSLRAEDTAVYYCAKEVGSPFDYWGQGTLVTVSS

SEQ ID NO: 70 - protein, 117 aa, Homo sapiens
EVQLLESGGGLVQPGGSLRLSCAASGFTFSSYAMSWVRQAPGKGLEWVSAISGSGGSTYYADSVKGRFTISRDNSKNTLYLQMNSLRAEDTAVYYCAKVLMVYADYWGQGTLVTVSS

SEQ ID NO: 71 - protein, 121 aa, Homo sapiens
EVQLLESGGGLVQPGGSLRLSCAASGFTFSSYAMNWVRQAPGKGLEWVSTISGSGDNTYYADSVKGRFTISRDNSKNTLYLQMNSLRAEDTAVYYCAKKFVLMVYAMLDYWGQGTLVTVSS

SEQ ID NO: 72 - protein, 121 aa, Homo sapiens
EVQLLESGGGLVQPGGSLRLSCAASGFTFSSYAMNWVRQAPGKGLEWVSTISGSGGNTYYADSVKGRFTISRDNSKNTLYLQMNSLRAEDTAVYYCAKKFVLMVYAMLDYWGQGTLVTVSS

SEQ ID NO: 73 - protein, 116 aa, Homo sapiens
QVQLVESGGGVVQPGRSLRLSCAASGFTFSSYGMHWVRQAPGKGLEWVAVIWYDGSNKYYADSVKGRFTISRDNSKNTLYLQMNSLRAEDTAVYYCARYYYGMDVWGQGTTVTVSS

SEQ ID NO: 74 - protein, 123 aa, Homo sapiens
QVQLVESGGGVVQPGRSLRLSCAASGFTFSSYGMHWVRQAPGKGLEWVAVIWYDGSDKYYADSVKGRFTISRDNSKNTLYLQMNSLRAEDTAVYYCARETGPLKLYYYGMDVWGQGTTVTVSS

SEQ ID NO: 75 - protein, 116 aa, Homo sapiens
QVQLVESGGGVVQPGRSLRLSCAASGFTFSSYGMHWVRQAPGKGLEWVAVIWYDGSNKYYADSVKGRFTISRDNSKNTLYLQMNSLRAEDTAVYYCARIAAGMDVWGQGTTVTVSS

SEQ ID NO: 76 - protein, 122 aa, Homo sapiens
QVHLVESGGGVVQPGRSLRLSCAASGFTFNSFGMHWVRQAPGKGLEWVALIWSDGSDKYYADSVKGRFTISRDNSKNTLYLQMNSLRAEDTAVYYCARAIAALYYYYGMDVWGQGTTVTVSS

SEQ ID NO: 77 - protein, 122 aa, Homo sapiens
QVQLVESGGGVVQPGRSLRLSCAASGFTFSSFGMHWVRQAPGKGLEWVALIWNDGSNKYYADSVKGRFTISRDNSKNTLYLQMNSLRAEDTAVYYCARAIAALYYYYGMDVWGHGTTVTVSS

SEQ ID NO: 78 - protein, 122 aa, Homo sapiens
QVQLVESGGGVVQPGRSLRLSCAASGFTFSSFGMHWVRQAPGKGLEWVALIWNDGSNKYYADSVKGRFTISRDNSKNTLYLQMNSLRAEDTAVYYCARAIAALYYYYGMDVWGQGTTVTVSS

SEQ ID NO: 79 - protein, 122 aa, Homo sapiens
QVHLVESGGGVVQPGRSLRLSCAASGFTFNSFGMHWVRQAPGKGLEWVALIWSDGSDEYYADSVKGRFTISRDNSKNTLYLQMNSLRAEDTAVYYCARAIAALYYYYGMDVWGQGTTVTVSS

SEQ ID NO: 80 - protein, 122 aa, Homo sapiens; identical to SEQ ID NO: 78

SEQ ID NO: 81 - protein, 122 aa, Homo sapiens
QVQLVESGGGVVQPGRSLRLSCAASGFTFSSYGMHWVRQAPGKGLEWVAIIWYDGSNKYYADSVKGRFTISRDNSKNTLYLQMNSLRAEDTAVYYCARRGGLAARPGGMDVWGQGTTVTVSS

SEQ ID NO: 82 - protein, 122 aa, Homo sapiens
QVQLVESGGGVVQPGRSLRLSCAASGFTFSSYGMHWVRQAPGKGLEWVAVIWYDGSNKYYADSVKGRFTISRDNSKNTLYLQMNSLRAEDTAVYYCARGIAVAYYYYGMDVWGQGTTVTVSS

SEQ ID NO: 83 - protein, 122 aa, Homo sapiens
QVQLVESGGGVVQPGRSLRLSCAASGFTFRSYGMHWVRQAPGKGLEWVALIWHDGSNTYYVDSVKGRFTISRDNSKNTLYLQMNSLRAEDTAVYYCARGIAVAYYYYGMDVWGQGTTVTVSS

SEQ ID NO: 84 - protein, 117 aa, Homo sapiens
QVQLQESGPGLVKPSQTLSLTCTVSGGSISSGGYYWSWIRQHPGKGLEWIGYIYYSGSTYYNPSLKSRVTISVDTSKNQFSLKLSSVTAADTAVYYCARYYYGMDVWGQGTTVTVSS

SEQ ID NO: 85 - protein, 122 aa, Homo sapiens
QVQLQESGPGLVKPSQTLSLTCTVSGGSISSSDYYWSWIRQHPGKGLEWIGYIYYSGSTYYNPSLKSRITISVDTSKNLFSLKLSSVTAADTAVYYCARGGVTTYYYAMDVWGQGTTVTVSS

SEQ ID NO: 86 - protein, 120 aa, Homo sapiens
QVQLQESGPGLVKPSQTLSLTCTVSGGSISSGGYYWSWIRQHPGKGLEWIGYIYYSGSTYYNPSLKSRVTISVDTSKNQFSLKLSSVTAADTAVYYCAREDTAMVYFDYWGQGTLVTVSS

SEQ ID NO: 87 - protein, 121 aa, Homo sapiens
QVQLQESGPGLVKPSQTLSLTCTVSGGSISSGGYYWSWIRQHPGKGLEWIGYIYNSGSTYYNPSLKSRVTISVDTSKNQFSLKLSSVTAADTAVYYCAREDTAMVPYFDYWGQGTLVTVSS

SEQ ID NO: 88 - protein, 115 aa, Homo sapiens
QVQLQQWGAGLLKPSETLSLTCAVYGGSFSGYYWSWIRQPPGKGLEWIGEINHSGSTNYNPSLKSRVTISVDTSKNQFSLKLSSVTAADTAVYYCARGQLVFDYWGQGTLVTVSS

SEQ ID NO: 89 - protein, 116 aa, Homo sapiens
QVQLQQWGAGLLKPSETLSLTCAVYGGSFSAYYWNWIRQPPGKGLEWIGEINHSGRTDYNPSLKSRVTISVDTSKKQFSLKLNSVTAADTAVYYCARGQLVPFDYWGQGTLVTVSS

SEQ ID NO: 90 - protein, 115 aa, Homo sapiens
QVQLQQSGPGLVKPSQTLSLTCAISGDSVSSNSAAWNWIRQSPSRGLEWLGRTYYRSKWYNDYAVSVKSRITINPDTSKNQFSLQLNSVTPEDTAVYYCARFDYWGQGTLVTVSS

SEQ ID NO: 91 - protein, 121 aa, Homo sapiens
QVQLQQSGPGLVKPSQTLSLTCAISGDSVSSNSAAWNWIRQSPSRGLEWLGRTYYRSKWYKNYSVSVKSRITINPDTSKNQFSLQLNSVTPGDTAVYYCARGGPTAAFDYWGQGTLVTVSS

SEQ ID NO: 92 - DNA, 345 bp, Homo sapiens
  source 1..345: mol_type = unassigned DNA
cagattcagctggtgcagtctggagctgaggtgaagaagcctggggcctcagtgaaggtctcctgcaaggcttctggttaccccttgaccagctatggtatcagctgggtgcgacaggcccctggacaagggcttgagtggatgggatggatcagcgcttacaatggtaacacaaactatgcacagaaggtccagggcagcgtcaccatgaccacagacacatccacgagcacagtctacatggagctgaggagcctgagatctgacgacacggccgtgtattactgtgcgagaggctacggtatggacgtctggggccaagggaccacggtcaccgtctcctct

SEQ ID NO: 93 - DNA, 327 bp, Homo sapiens
  source 1..327: mol_type = unassigned DNA
cagtctgccctgactcagcctgcctccgtgtctgggtctcctggacagtcgatcaccatctcctgcactggaaccagcagtgacgttggtggttataactctgtctcctggtaccaacagtacccaggcaaaccccccaaactcaagatttatgaggtcagtaatcggccctcaggggtttctaatcgcttctctggctccaagtctggcaacacggcctccctgaccatctctgggctccaggctgaggacgaggctgattatttctgcagctcatatacaagcaccagcatggtcttcggcggagggaccaagctgaccgtccta

SEQ ID NO: 94 - DNA, 345 bp, Homo sapiens
  source 1..345: mol_type = unassigned DNA
caggttcagctggtgcagtctggagctgaggtgaagaagcctggggcctcagtgaaggtctcctgcaaggcttctggttacaccttaaccagctatggtatcagctgggtgcgacaggcccctggacaagggcttgagtggatgggatgggtcagtttttataatggtaacacaaactatgcacagaagctccagggcagaggcaccatgaccacagacccatccacgagcacagcctacatggagctgaggagcctgagatctgacgacacggccgtgtattactgtgcgagaggctacggtatggacgtctggggccaagggaccacggtcaccgtctcctct

SEQ ID NO: 95 - DNA, 327 bp, Homo sapiens
  source 1..327: mol_type = unassigned DNA
cagtctgccctgactcagcctgcctccgtgtctgggtctcctggacagtcgatcaccatctcctgcactggaaccagcagtgacgttggtggttataactctgtctcctggtaccaacagcacccaggcaaagcccccaaactcatgatttatgaggtcagtaatcggccctcaggggtttctaatcgcttctctggctccaagtctggcaacacggcctccctgaccatctctgggctccaggctgaggacgaggctgattattactgcaattcatatacaagcaccagcatggtattcggcggagggaccaagctgaccgtccta

SEQ ID NO: 96 - DNA, 345 bp, Homo sapiens
  source 1..345: mol_type = unassigned DNA
caggttcagctggtgcagtctggagctgaagtgaagaagcctggggcctcagtgaaggtctcctgcaaggcttctggttacaccttgaccagctatggtatcagctgggtgcgacaggcccctggacaagggcttgagtggatgggatggatcagcttttacaatggtaacacaaactatgcacagaaggtccagggcagagtcaccatgaccacagacacatccacgagcacagtctacatggagctgaggagcctgagatctgacgacacggccgtgtattactgtgcgagaggctacggtatggacgtctggggccaagggaccacggtcaccgtctcctct

SEQ ID NO: 97 - DNA, 327 bp, Homo sapiens
  source 1..327: mol_type = unassigned DNA
cagtctgccctgactcagcctgcctccgtgtctgggtctcctggacagtcgatcaccatctcctgcactggaaccagcagtgacgttggtggttataactctgtctcctggtaccaacagcacccaggcaaaccccccaaactcatgatttatgaggtcagtaatcggccctcaggggtttctattcgcttctctggctccaagtctggcaacacggcctccctgaccatctctgggctccaggctgaggacgaggctgattatttctgcagctcatatacaagcaccagcatggtcttcggcggagggaccaagctgaccgtccta

SEQ ID NO: 98 - DNA, 345 bp, Homo sapiens
  source 1..345: mol_type = unassigned DNA
cagattcagctggtgcagtctggagctgaggtgaagaagcctggggcctcagtgaaggtctcctgcaaggcttctggttacaccttgaccagctatggtatcagctgggtgcgacaggcccctggacaagggcttgagtggatgggatggatcagcttttacaatggtaacacaaactatgcacagaaggtccagggcagagtcaccatgaccacagacacatccacgagcacagtctacatggagctgaggagcctgagatctgacgacacggccgtgtatttctgtgcgagaggttacggtatggacgtctggggccaagggaccacggtcaccgtctcctca

SEQ ID NO: 99 - DNA, 327 bp, Homo sapiens
  source 1..327: mol_type = unassigned DNA
cagtctgccctgactcagcctgcctccgtgtctgggtctcctggacagtcgatcaccatctcctgcactggaaccagcagtgacgttggtggttataactctgtctcgtggtaccaacagcacccaggcaaaccccccaaactcatgatttatgaggtcagtaatcggccctcaggggtttctaatcgcttctctggctccaagtctggcaacacggcctccctgaccatctctgggctccaggctgaggacgaggctgattatttctgcagctcatatacaagcaccagcatggtcttcggcggagggaccaagctggccgtccta

SEQ ID NO: 100 - DNA, 345 bp, Homo sapiens
  source 1..345: mol_type = unassigned DNA
caggttcagctggtgcagtctggagctgaggtgaagaagcctggggcctcagtgaaggtctcctgcaaggcttctggttacaccttaaccagctatggtatcagctgggtgcgacaggcccctggacaagggcttgagtggatgggatgggtcagtttttataatggtaacacaaactatgcacagaagctccagggcagaggcaccatgaccacagacccatccacgagcacagcctacatggagctgaggagcctgagatctgacgacacggccgtgtattactgtgcgagaggctacggtatggacgtctggggccaagggaccacggtcaccgtctcctca

SEQ ID NO: 101 - DNA, 327 bp, Homo sapiens
  source 1..327: mol_type = unassigned DNA
cagtctgccctgactcagcctgcctccgtgtctgggtctcctggacagtcgatcaccatctcctgcactggaaccagcagtgacgttggtggttataactctgtctcctggtaccaacagcacccaggcaaagcccccaaactcatgatttatgaggtcactaatcggccctcaggggtttctaatcgcttctctggctccaagtctggcaacacggcctccctgaccatctctgggctccaggctgaggacgaggctgattattactgcaactcatatacaagcaccagcatggtgttcggcggagggaccaagctgaccgtccta

SEQ ID NO: 102 - DNA, 363 bp, Homo sapiens
  source 1..363: mol_type = unassigned DNA
caggtgcagctgcaggagtcgggcccaggactggtgaagccttcacagaccctgtccctcacctgcactgtctctggtggctccatcagcagtggtggttactactggagctggatccgccagcacccagggaagggcctggagtggattgggtacatatataacagtgggagcacctactacaacccgtccctcaagagtcgagttaccatatcagtagacacgtctaagaaccagttctccctgaagctgagctctgtgactgccgcggacacggccgtgtattactgtgcgagagaggatacagctatggttccttactttgactactggggccagggaaccctggtcaccgtctcctca

SEQ ID NO: 103 - DNA, 333 bp, Homo sapiens
  source 1..333: mol_type = unassigned DNA
cagtctgtactgacgcagccgccctcagtgtctggggccccagggcagagggtcaccatctcctgcactgggagcagctccaacatcggggcacattatgatgtgcactggtaccagcaggttccaggaacagcccccaaactcctcatctatggtaacacctatcggccctcaggggtccctgaccgattctctggctccaagtctggcacctcagcctccctggccatcactgggctccaggctgaggatgaggctgattattactgccagtcctatgacaacagcctgagtggtgtggtattcggcggagggaccaagctgaccgtccta

SEQ ID NO: 104 - DNA, 366 bp, Homo sapiens
  source 1..366: mol_type = unassigned DNA
caggtgcacctggtggagtctgggggaggcgtggtccagcctgggaggtccctgagactctcctgtgcagcgtctggattcaccttcaacagctttggcatgcactgggtccgccaggctccaggcaaggggctggagtgggtggcacttatctggtctgatggaagtgatgaatactatgcagactccgtgaagggccgattcaccatctccagagacaattccaagaacacgctgtatctgcaaatgaacagcctgagagccgaggacacggctgtgtattactgtgcgagagccatagcagccctctactactactacggtatggacgtctggggccaagggaccacggtcaccgtctcctca

SEQ ID NO: 105 - DNA, 330 bp, Homo sapiens
  source 1..330: mol_type = unassigned DNA
cagtctgtgttgacgcagccgccctcagtgtctgcggccccaggacagaaggtcaccatctcctgctctggaagcagctccaacattgggaataattttgtatcctggtaccagcagctcccaggaacagcccccaaactcctcatttatgactataataagcgaccctcagggattcctgaccgattctctggctccaagtctggcacgtcagccaccctgggcatcaccggactccagactggggacgaggccgattattactgcggaacatgggatagcagcctgagtgcttatgtcttcggaactgggaccagggtcaccgtccta

SEQ ID NO: 106 - DNA, 366 bp, Homo sapiens
  source 1..366: mol_type = unassigned DNA
caggtgcagctggtggagtctgggggaggcgtggtccagcctgggaggtccctgagactctcctgtgcagcgtctggattcaccttcagcagctttggcatgcactgggtccgccaggctccaggcaaggggctggagtgggtggcacttatatggaatgatggaagtaataaatactatgcagactccgtgaagggccgattcaccatctccagagacaattccaagaacacgctgtatctgcaaatgaacagcctgagagccgaggacacggctgtgtattactgtgcgagagccatagcagccctctactactactacggtatggacgtctggggccaagggaccacggtcaccgtctcctca

SEQ ID NO: 107 - DNA, 330 bp, Homo sapiens
  source 1..330: mol_type = unassigned DNA
cagtctgtgttgacgcagccgccctcagtgtctgcggccccaggacagaaggtcaccatctcctgctctggaagcagctccaacattgggaataattttgtatcctggtaccagcagctcccaggaacagcccccaaactcctcatttatgactataataagcgaccctcagggattcctgaccgattctctggctccaagtctggcacgtcagccaccctgggcatcaccggactccagactggggacgaggccgattattactgcggaacatgggatagcagtctgagtggttatgtcttcggaactgggaccagggtcaccgtccta

SEQ ID NO: 108 - DNA, 366 bp, Homo sapiens
  source 1..366: mol_type = unassigned DNA
caggtgcacctggtggagtctgggggaggcgtggtccagcctgggaggtccctgagactctcctgtgcagcgtctggattcaccttcaacagctttggcatgcactgggtccgccaggctccaggcaaggggctggagtgggtggcacttatatggtctgatggaagtgataaatactatgcagactccgtgaagggccgattcaccatctccagagacaattccaagaacacgctgtatctgcaaatgaacagcctgagagccgaggacacggctgtgtattactgtgcgagagccatagcagccctctactactactacggtatggacgtctggggccaagggaccacggtcaccgtctcctca

SEQ ID NO: 109 - DNA, 330 bp, Homo sapiens
  source 1..330: mol_type = unassigned DNA
cagtctgtgttgacgcagccgccctcagtgtctgcggccccaggacagaaggtcaccatctcctgctctggaagcagttccaacattgggaataattttgtatcctggtaccagcagttcccaggaacagcccccaaactcctcatttatgactataataagcgaccctcagggattcctgaccgattctctggctccaagtctggcacgtcagccaccctgggcatcaccggactccagactggggacgaggccgattattactgcggaacatgggatagcagcctgagttcttatgtcttcggaactgggaccagggtcaccgtccta

SEQ ID NO: 110 - DNA, 366 bp, Homo sapiens
  source 1..366: mol_type = unassigned DNA
caggtgcagctggtggagtctgggggaggcgtggtccagcctgggaggtccctgagactctcctgtgcagcgtctggattcaccttcagcagctttggcatgcactgggtccgccaggctccaggcaaggggctggagtgggtggcacttatatggaatgatggaagtaataaatactatgcagactccgtgaagggccgattcaccatctccagagacaattccaagaacacgctgtatctgcaaatgaacagcctgagagccgaggacacggctgtgtattactgtgcgagagccatagcagccctctactactactacggtatggacgtctggggccacgggaccacggtcaccgtctcctca

SEQ ID NO: 111 - DNA, 330 bp, Homo sapiens
  source 1..330: mol_type = unassigned DNA
cagtctgtgttgacgcagccgccctcagtgtctgcggccccaggacagaaggtcaccatctcctgctctggaagcagctccaacattgggaataattttgtatcctggtaccagcagctcccaggaacagcccccaaactcctcatttatgactataataagcgaccctcagggattcctgaccgattctctggctccaagtctggcacgtcagccaccctgggcatcaccggactccagactggggacgaggccgattattactgcggaacatgggatagcagcctgagtggttatgtcttcggaactgggaccagggtcaccgtccta

SEQ ID NO: 112 - DNA, 366 bp, Homo sapiens; identical to SEQ ID NO: 106
  source 1..366: mol_type = unassigned DNA

SEQ ID NO: 113 - DNA, 330 bp, Homo sapiens
  source 1..330: mol_type = unassigned DNA
cagtctgtgttgacgcagccgcccacagtgtctgcggccccaggacagaaggtcaccatctcctgctctggaagcagctccaacattgggaataattttgtatcctggtaccagcagctcccaggaacagcccccaaactcctcatttatgactataataagcgaccctcagggattcctgaccgattctctggctccaagtctggcacgtcagccaccctgggcatcaccggactccagactggggacgaggccgattactactgcggaacatgggatagcagcctgagtggttatgtcttcggaactgggaccagggtcaccgtccta

SEQ ID NO: 114 - DNA, 366 bp, Homo sapiens
  source 1..366: mol_type = unassigned DNA
caggtgcagctggtggagtctgggggaggcgtggtccagcctgggaggtccctgagactctcctgtgcagcgtctggattcaccttcaggagctatggcatgcactgggtccgccaggctccaggcaaggggctggagtgggtggcacttatatggcatgatggaagtaatacatactatgtagactccgtgaagggccgattcaccatctccagagacaattccaagaacacgctgtatctgcaaatgaacagcctgagagccgaggacacggctgtgtattactgtgcgagaggtatagcagtggcttactactactacggtatggacgtctggggccaagggaccacggtcaccgtctcctca

SEQ ID NO: 115 - DNA, 330 bp, Homo sapiens
  source 1..330: mol_type = unassigned DNA
cagtctgtgttgacgcagccgccctcagtgtctgcggccccaggacagaaggtcaccatctcctgctctggaagcagctccaacattgggaataattttgtatcctggtaccagcagctcccaggaacagcccccaaactcctcatttatgacagtaataagcgaccctcagggattcctgaccgattctctggctccaagtctggcacgtcagccaccctggacatcaccggactccagactggggacgaggccgattattactgcggaacatgggatagcagcctgagtgcttatgttttcggaactgggaccaaggtcaccgtccta

SEQ ID NO: 116 - DNA, 363 bp, Homo sapiens
  source 1..363: mol_type = unassigned DNA
gaggtgcagctgttggagtctgggggaggcttggtacagcctggggggtccctgagactctcctgtgcagcctctggattcacctttagcagctatgccatgaactgggtccgccaggctccagggaaggggctggagtgggtctcaactattagtggtagtggtgataacacatactacgcagactccgtgaagggccggttcaccatctccagagacaattccaagaacacgctgtatctgcaaatgaacagcctgagagccgaggacacggccgtatattactgtgcgaaaaagtttgtactaatggtgtatgctatgcttgactactggggccagggaaccctggtcaccgtctcctca

SEQ ID NO: 117 - DNA, 321 bp, Homo sapiens
  source 1..321: mol_type = unassigned DNA
gacatcctgatgacccagtctccatcctccctgtctgcatctgttggagacagagtcaccatcacttgccgggcaagtcagagcattagcagttatttaaattggtatcagcagaaaccagggaaagcccctaaggtcctgatctatgctgcctccagtttgcaaagtggggtcccatcaaggttcagtggcagtggatctgggacagatttcactctcaccatcaacagtctgcaacctgaagattttgcaacttactactgtcaacagagttacagttcccccatcaccttcggccaagggacacgactggagattaaa

SEQ ID NO: 118 - DNA, 363 bp, Homo sapiens
  source 1..363: mol_type = unassigned DNA
gaggtgcagctgttggagtctgggggaggcttggtacagccgggggggtccctgagactctcctgtgcagcctctggattcacctttagcagctatgccatgaactgggtccgccaggctccagggaaggggctggagtgggtctcaactattagtggtagtggtggtaacacatactacgcagactccgtgaagggccggttcaccatctccagagacaattccaagaacacgctgtatctgcaaatgaacagcctgagagccgaggacacggccgtatattactgtgcgaaaaagtttgtactaatggtgtatgctatgcttgactactggggccagggaaccctggtcaccgtctcctca

SEQ ID NO: 119 - DNA, 321 bp, Homo sapiens
  source 1..321: mol_type = unassigned DNA
gacatccagatgacccagtctccatcctccctatctgcatctgtaggagacagagtcaccatcacttgccgggcaagtcagagcattagcatctatttaaattggtatcagcagaagccagggaaagccccttacctcctgatctatgctgcagccagtttgcaaagtggggtcccatcaaggttcagtggcagtggatctgggacagatttcactctcaccatcagcagtctgcaacctgaagattttgcaacttactactgtcaacagagttacagtgcccccatcaccttcggccaagggacacgactggagattaaa

SEQ ID NO: 120 - DNA, 345 bp, Homo sapiens
  source 1..345: mol_type = unassigned DNA
caggttcagctggtgcagtctggagctgaggtgaagaagcctggggcctcactgaaggtctcctgcaaggcttctggttacagtttgaccagctatggtatcagctgggtgcgacaggcccctggacaagggcttgagtggatgggatggatcagcgcttacaatggtaacacaaactatgcacagaaggtccagggcagagtcaccatgaccacagacacatccacgagcacagtctacatggaggtgaggagtctgagatctgacgacacggccgtgtattactgtgcgagaggctacggtatggacgtctggggccaagggaccacggtcaccgtctcctca

SEQ ID NO: 121 - DNA, 327 bp, Homo sapiens
  source 1..327: mol_type = unassigned DNA
cagtctgccctgactcagcctgcctccgtgtctgggtctcctggacagtcgatcaccatctcctgcactggaaccagcagtgacgttggtggttataactctgtctcctggtaccaacagcacccaggcaaaccccccaaactcatgatttatgaggtcagtaatcggccctcaggggtttctaatcgcttctctggctccaagtctggcaatacggcctccctgaccatctctgggctccaggctgaggacgaggctgattatttctgcagctcatatacaagcaccagcatggtcttcggcggagggaccaagctgaccgtccta

SEQ ID NO: 122 - DNA, 345 bp, Homo sapiens
  source 1..345: mol_type = unassigned DNA
caggttcagctggtgcagtctggagctgaggtgaagaggcctggggcctcagtgaaggtctcctgcaaggcttctggttacaccttgaccagctatggtatcagctgggtgcgacaggcccctggacaagggcttgagtggatgggatggatcagcgtttacaatggtaacacaaactatgcacagaaggtccagggcagagtcaccatgaccacagacacatccacgagcacagtctacatggagctgaggagcctgagctctgacgacacggccgtgtattactgtgcgagaggctacggtatggacgtctggggccaagggaccacggtcaccgtctcctca

SEQ ID NO: 123 - DNA, 327 bp, Homo sapiens; identical to SEQ ID NO: 97
  source 1..327: mol_type = unassigned DNA

SEQ ID NO: 124 - DNA, 345 bp, Homo sapiens
  source 1..345: mol_type = unassigned DNA
caggttcagctggtgcagtctggagctgaggtgaagaagcctggggcctcagtgaaggtctcctgcaaggcttctggttaccccttgaccagctatggtatcagctgggtgcgacaggcccctggacaagggcttgagtggatgggatggatcagcgcttacaatggtaacacaaactatgcacagaaggtccagggcagagtcaccatgaccacagacacatccacgagcacagtctacatggagttgaggagcctgagatctgacgacacggccgtgtattactgtgcgagaggctacggtatggacgtctggggccaagggaccacggtcaccgtctcctca

SEQ ID NO: 125 - DNA, 327 bp, Homo sapiens; identical to SEQ ID NO: 121
  source 1..327: mol_type = unassigned DNA

SEQ ID NO: 126 - DNA, 345 bp, Homo sapiens
  source 1..345: mol_type = unassigned DNA
caggttcagttggtgcagtctggagctgaggtgaagaagcctggggcctcagtgaaggtctcctgcaaggcttctggttacgccttgaccagctatggtatcagctgggtgcgacaggcccctggacaagggcttgagtggatgggatggatcagcgcttacaatggtaacacaaactatgcacagaaggtccagggcagagtcaccatgaccacagacacatccacgagcacagtctacatggagctgaggagcctgagatctgacgacacggccgtgtattactgtgcgagaggctacggtatggacgtctggggccaagggaccacggtcaccgtctcctca

SEQ ID NO: 127 - DNA, 327 bp, Homo sapiens
  source 1..327: mol_type = unassigned DNA
cagtctgccctgactcagcctgcctccgtgtctgggtctcctggacagtcgatcaccatctcctgcactggaaccaacagtgacgttggtggttataactctgtctcctggtaccaacagcacccaggcaaaccccccaaactcatgatttatgaggtcagtaatcggccctcagggatttctaatcgcttctctggctccaagtctggcaacacggcctccctgaccatctctgggctccaggctgaggacgaggctgattatttctgcagctcatatacaagcaccagcatggtcttcggcggagggaccaagctgaccgtccta

SEQ ID NO: 128 - DNA, 345 bp, Homo sapiens
  source 1..345: mol_type = unassigned DNA
caggttcagctggtgcagtctggagctgaggtgaagaagcctggggcctcagtgaaggtctcctgcaaggcttctggttacagctttaccagctatggtatcagctgggtgcgacaggcccctggacaagggcttgagtggatgggatgggtcagcgcttacaatggtaacacaaactatgcacagaagttccagggcagagtcaccatgaccacagacacatccacgagcacagcctacatggaactgaggagcctgagatctgacgacacggccgtgtattactgtgcgagaggctacgttatggacgtctggggccaagggaccacggtcaccgtctcctca

SEQ ID NO: 129 - DNA, 327 bp, Homo sapiens
  source 1..327: mol_type = unassigned DNA
cagtctgccctgactcagcctgcctccgtttctgggtctcctggacagtcgatcaccatctcctgcactggaaccagcagtgacgttggtgcttataactctgtctcctggtaccaacagcacccaggcaaagcccccaaacgcatgatttatgaggtcagtaatcggccctcaggggtttctaatcgcttctctggctccaagtctggcaacacggcctccctgaccatctctgggctccaggctgaggacgaggctgattattactgcagctcatatacaagcaccaacatggtattcggcggagggaccaagctgaccgtccta

SEQ ID NO: 130 - DNA, 363 bp, Homo sapiens
  source 1..363: mol_type = unassigned DNA
caggtacagttgcagcagtcaggtccaggactggtgaagccctcgcagaccctctcactcacctgtgccatctccggggacagtgtctctagcaacagtgctgcttggaactggatcaggcagtccccatcgagaggccttgagtggctgggaaggacatactacaggtccaagtggtataaaaattattcagtatctgtgaaaagtcgaataaccatcaacccagacacatccaagaaccagttctctctgcaactgaactctgtgactcccggggacacggctgtgtattactgtgcaagaggggggccaactgctgcttttgactactggggccagggaaccctggtcaccgtctcctca

SEQ ID NO: 131 - DNA, 330 bp, Homo sapiens
  source 1..330: mol_type = unassigned DNA
ctttctgccctgactcagcctgcctccgtgtctgggtctcctggacagtcgatcaccatctcctgcactggaaccagcagtgatgttgggaattataaccttgtctcctggtaccaacagtattcaggcaaagcccccaaactcatgatttatgaggtcagtaagcggccctcaggggtttctaatcgcttctctggctccaagtctggcaacacggcctccctgacaatctctgggctccaggctgaggacgaggctgattattactgctgctcatatgcaggtagtagcactttggttttcggcggagggaccaagctgaccgtccta

SEQ ID NO: 132 - DNA, 357 bp, Homo sapiens
  source 1..357: mol_type = unassigned DNA
gaggtgcagttggtggagtctgggggaggcttggtccagcctggggggtccctgagactctcctgtgtagtctctggattcacctttagtagctattggatgagctgggtccgccaggctccagggaaggggctggagtgggtggccaacataaagcaagatggaagtgagaaatactatgtggactctgtgaagggccgattcaccatctccagagacaacgccaagaactcactgtatctgcaaatgaacagcctgagagccgaggacacggctgtatattactgtgcgagagagtcaaactggggatttgcttttgatatctggggccaagggacaatggtcaccgtctcttca

SEQ ID NO: 133 - DNA, 327 bp, Homo sapiens
  source 1..327: mol_type = unassigned DNA
cagtctgtgctgactcagccaccctcagcgtctgggacccccgggcagagggtcaccatctcttgttctggaagcagctccaacatcggaagtaagactgtaaactggtaccaacaggtcccaggaacggcccccaaactcctcatctataggaataatcagcggcccttaggggtccctgaccgattctctggctccaagtctggcacctcagcctccctggccatcagtgggctccagtctgaggatgaggctgattattattgtgcagcatgggatgacagcctgaattgggtgttcggcggagggaccaagctgaccgtccta

SEQ ID NO: 134 - DNA, 357 bp, Homo sapiens
  source 1..357: mol_type = unassigned DNA
gaggtgcagctggtggagtctgggggaggcttggtccagcctggggggtccctgagactctcctgtgcagcctctggattcacctttagtcgctattggatgagctgggtccgccaggctccagggaaggggctggagtgggtggccaacataaagcatgatggaagtgagaaatactatgtggactctgtgaagggccgattcaccatttccagagacaacgccaagaactcactgtatctgcaaatgaacagcctgagagccgaggacacggctgtgtattactgtgcgagagagtcaaactggggatttgcttttgatgtctggggccacgggacaatggtcaccgtctcttca

SEQ ID NO: 135 - DNA, 327 bp, Homo sapiens
  source 1..327: mol_type = unassigned DNA
cagtctgtgctgactcagccaccctcagcgtctgggccccccggacagagggtcaccatctcttgttctggaagcagctccaacatcggaagtaatactgtaaactggtaccagcagctcccaggaacggcccccaaactcctcatctatagtaataatcggcggccctcaggggtccctgaccgattctctggctccaagtctggcacctcagcctccctggccatcagtgggctccagtctgaggatgaggctgattattactgtgcagcatgggatgacagcctgaattgggtgttcggcggagggaccaagctgaccgtccta

SEQ ID NO: 136 - DNA, 351 bp, Homo sapiens
  source 1..351: mol_type = unassigned DNA
gaggtgcagctgttggagtctgggggaggcttggtacagcctggggggtccctgagactctcctgtgcagcctctggattcacctttagcagctatgccatgagctgggtccgccaggctccagggaaggggctggagtgggtctcaactattagtggtagtggtggtaggacatattacgcagactccgtgaagggccggttcaccatctccagagacaattccaagaacacgctgtatctgcaaatgaacagcctgagagccgaggacacggccgtatattactgtgcgaaagaagttggcagtccctttgactactggggccagggaaccctggtcaccgtctcctca

SEQ ID NO: 137 - DNA, 330 bp, Homo sapiens
  source 1..330: mol_type = unassigned DNA
cagtctgtgttgacgcagccgccctcagtgtctgcggccccaggacagaaggtcaccatctcctgctctggaagcaactccaacattgggaataattatgtatcctggtaccagcagctcccaggaacagcccccaaactcctcatttatgacaataataagcgaccctcagggattcctgaccgattctctggctccaactctggcacgtcagccaccctgggcatcaccggactccagactggggacgaggccgattattactgcggaacatgggatagcagcctgagtgctgtggtattcggcggagggaccaagctgaccgtccta

SEQ ID NO: 138 - DNA, 366 bp, Homo sapiens
  source 1..366: mol_type = unassigned DNA
caggtgcagctggtggagtctgggggaggcgtggtccagcctgggaggtccctgagactctcctgtgcagcgtctggattcaccttcagtagctatggcatgcactgggtccgccaggctccaggcaaggggctggagtgggtggcaattatatggtatgatggaagtaataaatactatgcagactccgtgaagggccgattcaccatctccagagacaattccaagaacacactgtatcttcaaatgaacagcctgagagccgaggacacggctgtgtattactgtgcgaggagggggggtctggcagctcgtccgggcggtatggacgtctggggccaagggaccacggtcaccgtctcctca

SEQ ID NO: 139 - DNA, 318 bp, Homo sapiens
  source 1..318: mol_type = unassigned DNA
tcctatgagctgactcagccaccctcagtgtctgtgtccccaggacagacagccagaatcacctgctctggagataaattgggggataaatatgcttgctggtatcagcagaaaccaggccagtcccctgtgctggtcatctatcaaaataccaagtggcccttagggatccctgagcgattctctggctccaagtctgggaacacagtcactctgaccatcagcgggacccaggctatggatgaggctgactattactgtcaggcgtgggacagcagcactgtggtattcggcggagggaccaagctgaccgtccta

SEQ ID NO: 140 - DNA, 366 bp, Homo sapiens
  source 1..366: mol_type = unassigned DNA
caggtgcagctgcaggagtcgggcccaggactggtgaagccttcacagaccctgtccctcacctgcactgtctctggtggctccatcagcagtagtgattactactggagctggatccgccagcacccagggaagggcctggagtggattgggtacatctattacagtgggagcacctactacaacccgtccctcaagagtcgaattaccatatcagtagacacgtctaagaacctgttctccctgaagttgagctctgtgactgccgcggacacggccgtgtattactgtgcgagagggggggtgactacgtactactacgctatggacgtctggggccaagggaccacggtcaccgtctcctca

SEQ ID NO: 141 - DNA, 321 bp, Homo sapiens
  source 1..321: mol_type = unassigned DNA
gacatacagatgacccagtctccatcctccctgtctgcatctgtaggagacagagtcaccatcacttgccgggcaagtcagcgcattagcaactatttaagttggtatctgcagaaaccagggattgcccctaagctcctgatctatgctgcatccagtttgcagagtggggtcccatcaaggttcagtggcagtggatctgggacagatttcactctcaccatcagcagtctgcaatctgaagattttgcaacttactactgtcaacagagttacagtaccccgctcattttcggcggagggaccaaggtggagatcaaa

SEQ ID NO: 142 - DNA, 369 bp, Homo sapiens
  source 1..369: mol_type = unassigned DNA
caggtgcagctggtggagtctgggggaggcgtggtccagcctgggaggtccctgagactctcctgtgcagcgtctggattcaccttcagtagctatggcatgcactgggtccgccaggctccaggcaaggggctggagtgggtggcagttatatggtatgatggaagtgataaatactatgcagactccgtgaagggccgattcaccatctccagagacaattccaagaacacgctgtatctgcaaatgaacagcctgagagccgaggacacggctgtgtattactgtgcgagagagactggtcccttgaaactctactactacggtatggacgtctggggccaagggaccacggtcaccgtctcctca

SEQ ID NO: 143 - DNA, 336 bp, Homo sapiens
  source 1..336: mol_type = unassigned DNA
gatattgtgatgactcagtctccactctccctgtccgtcacccctggagagccgccctccatctcctgcaggtctagtcagagcctcctgcatagtaatggatacaactttttgaattggtacctgcagaagccagggcagtctccacaactcctgatctatttgggttctcatcgggcctccggggtccctgacaggttcagtggcagtggatcaggcacagattttacactggaaatcagcagagtggaggctgaggatgttggggtttattactgcatgcaagttctacaaactccattcactttcggccctgggaccaaagtggatatcaaa

SEQ ID NO: 144 - DNA, 357 bp, Homo sapiens
  source 1..357: mol_type = unassigned DNA
gaggtgcagctggtggagtctgggggaggcttggtccagcctggggggtccctgagactctcctgtgcagcctctggactcacctttagtaacttttggatgagctgggtccgccaggctccagggaaggggctggagtgggtggccaacataaagcaagatggaagtgagaaatactatgtggactctgtgaagggccgattcaccatctccagagacaacgccaagaattcactgtatctgcaaatgaacagcctgagagccgaggacacggctgtgtattcctgtacgagagagtcaaactggggatttgcttttgatatctggggccaagggacaatggtcaccgtctcttca

SEQ ID NO: 145 - DNA, 327 bp, Homo sapiens
  source 1..327: mol_type = unassigned DNA
cagtctgtgctgactcagccaccctcagcgtctgggacccccgggcagagggtcaccatctcttgttctggaagcagctccaacatcggaagtaaaactgtaaactggtaccagcagttcccaggaacggcccccaaactcctcatctatagtaataatcggcggccctcaggggtccctgaccgattctctggctccaagtctggcacctcagcctccctggccatcagtgggctccagtctgaggatgaggctgattattactgtgcagcatgggatgacagcctgaattgggtgttcggcgcagggaccaagctgaccgtccta

SEQ ID NO: 146 - DNA, 345 bp, Homo sapiens
  source 1..345: mol_type = unassigned DNA
caggttcagctggtgcagtctggagctgaggtgaagaagcctggggcctcagtgaaggtctcctgcaaggcttctggttacacctttaccagctatggtatcagctgggtgcgacaggcccctggacaagggcttgagtggatgggatggatcagcacttacaatggtaacacaaactatgcacagaaggtccagggcagagtcaccatgaccacagacacatccacgagcacagcctacatggagctgaggagcctgagatctgacgacacggccgtttattactgtgcgagagggtatactcgggactactggggccagggaaccctggtcaccgtctcctca

SEQ ID NO: 147 - DNA, 348 bp, Homo sapiens
  source 1..348: mol_type = unassigned DNA
cagcctgtgctgactcagccactttttgcatcagcctccctgggagcctcggtcacactcacctgcaccctgagcagcggctacagtagttatgaagtggactggtatcagcagagaccagggaagggcccccggtttgtcatgcgagtggacactggtgggattgtgggatccaagggggaaggcatccctgatcgcttctcagttttgggctcaggcctgaatcggtatctgaccatcaagaacatccaggaagaggatgagagtgactaccactgtggggcagaccatggcagtgggaccaacttcgtggtggtattcggcggagggaccaagctgaccgtccta

SEQ ID NO: 148 - DNA, 348 bp, Homo sapiens
  source 1..348: mol_type = unassigned DNA
caggtgcagctacagcagtggggcgcaggactgttgaagccttcggagaccctgtccctcacctgcgctgtctatggtgggtccttcagtgcgtactactggaactggatccgccagcccccagggaaggggctggagtggattggggaaatcaatcatagtggaagaaccgactacaacccgtccctcaagagtcgagtcaccatatcagtagacacgtccaagaagcagttctccctgaagctgaactctgtgaccgccgcggacacggctgtgtattactgtgcgagagggcagctcgtcccctttgactactggggccagggaaccctggtcaccgtctcttca

SEQ ID NO: 149 - DNA, 330 bp, Homo sapiens
  source 1..330: mol_type = unassigned DNA
cagtctgtgctgactcagccaccctcagcgtctgggacccccgggcagagggtcaccatctcttgttctggaagcagctccaacatcggaagtaatactgtaaattggtatcagcaactcccaggaacggcccccaaactcctcatctatagtaataatcagcggccctcaggggtccctgaccgattctctggctccaagtctggcacctcagcctccctggccatcagtgggctccagtctgaggatgaggctgattattactgtgcagtatgggatgacagcctgaatggttgggtgttcggcggagggaccaagctgaccgtccta

SEQ ID NO: 150 - DNA, 345 bp, Homo sapiens
  source 1..345: mol_type = unassigned DNA
caggttcagctggtgcagtctggagctgaggtgaagaagcctggggcctcagtgaaggtctcctgcaaggcttctggttacacctttcccagctatggtatcagctgggtgcgacaggcccctggacaagggcttgagtggatgggatggatcagcgcttacaatggtaacacaaactatgcagagaagctccagggcagagtcaccatgaccacagacacatccacgagcacagcctacatggaggtgaggagcctgagatctgacgacacggccgtgttttactgtgcgagaggctacgttatggacgtctggggccaagggaccacggtcaccgtctcctct

SEQ ID NO: 151 - DNA, 327 bp, Homo sapiens
  source 1..327: mol_type = unassigned DNA
cagtctgccctgactcagcctgcctccgtgtctgggtctcctggacagtcgatcaccatctcctgcactggaaccagcagtgacgttggtcgttataattctgtctcctggtaccaacaccacccaggcaaagcccccaaagtcatgatttatgaggtcagtaatcggccctcaggggtttctactcgcttctctggctccaagtctggcaacacggcctccctgaccatctctgggctccaggctgaggacgaggctgattattactgcagctcatatacaagcagcagcgttgtattcggcggagggaccaaactgaccgtccta

SEQ ID NO: 152 - DNA, 369 bp, Homo sapiens
  source 1..369: mol_type = unassigned DNA
gaggtgcagctggtggagtctgggggaggcctggtcaagcctggggggtccctgagactctcctgtgcagcctctggattcaccttcagtagctatagcatgaactgggtccgccaggctccagggaaggggctggagtgggtctcatccattagtagtagtagtagttacatttcctacgcagactcagtgaagggccgattcaccatctccagagacaacgccaagaactcactgtatctgcaaatgaacagcctgagagccgaggacacggctgtgtatttctgtgcgagagattacgatttttggagtgcttactatgatgcttttgatgtctggggccaagggacaatggtcaccgtctcttca

SEQ ID NO: 153 - DNA, 333 bp, Homo sapiens
  source 1..333: mol_type = unassigned DNA
cagtctgtgctgacgcagccgccctcagtgtctggggccccagggcagagggtcaccatctcctgcactgggagcagctccaacatcggggcaggttatgatgtacactggtaccagcagcttccaggaacagcccccaaactcctcatctctggtaacagcaatcggccctcaggggtccctgaccgattctctggctccaagtctggcacctcagcctccctggccatcactgggctccaggctgaggatgaggctgattattactgccagtcctatgacagcagcctgagtggttcggtattcggcggagggaccaagctgaccgtccta

SEQ ID NO: 154 - protein, 326 aa, Homo sapiens
ASTKGPSVFPLAPCSRSTSESTAALGCLVKDYFPEPVTVSWNSGALTSGVHTFPAVLQSSGLYSLSSVVTVPSSNFGTQTYTCNVDHKPSNTKVDKTVERKCCVECPPCPAPPVAGPSVFLFPPKPKDTLMISRTPEVTCVVVDVSHEDPEVQFNWYVDGVEVHNAKTKPREEQFNSTFRVVSVLTVVHQDWLNGKEYKCKVSNKGLPAPIEKTISKTKGQPREPQVYTLPPSREEMTKNQVSLTCLVKGFYPSDIAVEWESNGQPENNYKTTPPMLDSDGSFFLYSKLTVDKSRWQQGNVFSCSVMHEALHNHYTQKSLSLSPGK

SEQ ID NO: 155 - protein, 327 aa, Homo sapiens
ASTKGPSVFPLAPCSRSTSESTAALGCLVKDYFPEPVTVSWNSGALTSGVHTFPAVLQSSGLYSLSSVVTVPSSSLGTKTYTCNVDHKPSNTKVDKRVESKYGPPCPSCPAPEFLGGPSVFLFPPKPKDTLMISRTPEVTCVVVDVSQEDPEVQFNWYVDGVEVHNAKTKPREEQFNSTYRVVSVLTVLHQDWLNGKEYKCKVSNKGLPSSIEKTISKAKGQPREPQVYTLPPSQEEMTKNQVSLTCLVKGFYPSDIAVEWESNGQPENNYKTTPPVLDSDGSFFLYSRLTVDKSRWQEGNVFSCSVMHEALHNHYTQKSLSLSLGK

SEQ ID NO: 156 - protein, 105 aa, Homo sapiens
QPKAAPSVTLFPPSSEELQANKATLVCLISDFYPGAVTVAWKADSSPVKAGVETTTPSKQSNNKYAASSYLSLTPEQWKSHRSYSCQVTHEGSTVEKTVAPTECS

SEQ ID NO: 157 - protein, 106 aa, Homo sapiens
TVAAPSVFIFPPSDEQLKSGTASVVCLLNNFYPREAKVQWKVDNALQSGNSQESVTEQDSKDSTYSLSSTLTLSKADYEKHKVYACEVTHQGLSSPVTKSFNRGEC

SEQ ID NO: 158 - protein, 14 aa, Homo sapiens
TGTSSDVGGYNSVS

SEQ ID NO: 159 - protein, 14 aa, Homo sapiens
TGTNSDVGGYNSVS

SEQ ID NO: 160 - protein, 14 aa, Homo sapiens
TGTSSDVGAYNSVS

SEQ ID NO: 161 - protein, 14 aa, Homo sapiens
TGTSSDVGRYNSVS

SEQ ID NO: 162 - protein, 7 aa, Homo sapiens
EVSNRPS

SEQ ID NO: 163 - protein, 7 aa, Homo sapiens
EVTNRPS

SEQ ID NO: 164 - protein, 9 aa, Homo sapiens
SSYTSTSMV

SEQ ID NO: 165 - protein, 9 aa, Homo sapiens
NSYTSTSMV

SEQ ID NO: 166 - protein, 9 aa, Homo sapiens
SSYTSTNMV

SEQ ID NO: 167 - protein, 9 aa, Homo sapiens
SSYTSSSVV

SEQ ID NO: 168 - protein, 10 aa, Homo sapiens
GYPLTSYGIS

SEQ ID NO: 169 - protein, 10 aa, Homo sapiens
GYSLTSYGIS

SEQ ID NO: 170 - protein, 10 aa, Homo sapiens
GYALTSYGIS

SEQ ID NO: 171 - protein, 10 aa, Homo sapiens
GYTLTSYGIS

SEQ ID NO: 172 - protein, 10 aa, Homo sapiens
GYSFTSYGIS

SEQ ID NO: 173 - protein, 10 aa, Homo sapiens
GYTFPSYGIS

SEQ ID NO: 174 - protein, 17 aa, Homo sapiens
WISAYNGNTNYAQKVQG

SEQ ID NO: 175 - protein, 17 aa, Homo sapiens
WVSFYNGNTNYAQKLQG

SEQ ID NO: 176 - protein, 17 aa, Homo sapiens
WISFYNGNTNYAQKVQG

SEQ ID NO: 177 - protein, 17 aa, Homo sapiens
WISVYNGNTNYAQKVQG

SEQ ID NO: 178 - protein, 17 aa, Homo sapiens
WVSAYNGNTNYAQKFQG

SEQ ID NO: 179 - protein, 17 aa, Homo sapiens
WISAYNGNTNYAEKLQG

SEQ ID NO: 180 - protein, 6 aa, Homo sapiens
GYGMDV

SEQ ID NO: 181 - protein, 6 aa, Homo sapiens
GYVMDV

SEQ ID NO: 182 - protein, 13 aa, Homo sapiens
SGSSSNIGNNFVS

SEQ ID NO: 183 - protein, 7 aa, Homo sapiens
DYNKRPS

SEQ ID NO: 184 - protein, 7 aa, Homo sapiens
DSNKRPS

SEQ ID NO: 185 - protein, 11 aa, Homo sapiens
GTWDSSLSGYV

SEQ ID NO: 186 - protein, 11 aa, Homo sapiens
GTWDSSLSAYV

SEQ ID NO: 187 - protein, 11 aa, Homo sapiens
GTWDSSLSSYV

SEQ ID NO: 188 - protein, 10 aa, Homo sapiens
GFTFSSFGMH

SEQ ID NO: 189 - protein, 10 aa, Homo sapiens
GFTFNSFGMH

SEQ ID NO: 190 - protein, 10 aa, Homo sapiens
GFTFRSYGMH

SEQ ID NO: 191 - protein, 17 aa, Homo sapiens
LIWNDGSNKYYADSVKG

SEQ ID NO: 192 - protein, 17 aa, Homo sapiens
LIWSDGSDEYYADSVKG

SEQ ID NO: 193 - protein, 17 aa, Homo sapiens
LIWSDGSDKYYADSVKG

SEQ ID NO: 194 - protein, 17 aa, Homo sapiens
LIWHDGSNTYYVDSVKG

SEQ ID NO: 195 - protein, 13 aa, Homo sapiens
AIAALYYYYGMDV

SEQ ID NO: 196 - protein, 13 aa, Homo sapiens
GIAVAYYYYGMDV

SEQ ID NO: 197 - protein, 13 aa, Homo sapiens
SGSSSNIGSNTVN

SEQ ID NO: 198 - protein, 13 aa, Homo sapiens
SGSSSNIGSKTVN

SEQ ID NO: 199 - protein, 7 aa, Homo sapiens
SNNRRPS

SEQ ID NO: 200 - protein, 7 aa, Homo sapiens
RNNQRPL

SEQ ID NO: 201 - protein, 10 aa, Homo sapiens
AAWDDSLNWV

SEQ ID NO: 202 - protein, 10 aa, Homo sapiens
GFTFSRYWMS

SEQ ID NO: 203 - protein, 10 aa, Homo sapiens
GLTFSNFWMS

SEQ ID NO: 204 - protein, 10 aa, Homo sapiens
GFTFSSYWMS

SEQ ID NO: 205 - protein, 17 aa, Homo sapiens
NIKHDGSEKYYVDSVKG

SEQ ID NO: 206 - protein, 17 aa, Homo sapiens
NIKQDGSEKYYVDSVKG

SEQ ID NO: 207 - protein, 10 aa, Homo sapiens
ESNWGFAFDV

SEQ ID NO: 208 - protein, 10 aa, Homo sapiens
ESNWGFAFDI

SEQ ID NO: 209 - protein, 11 aa, Homo sapiens
RASQSISSYLN

SEQ ID NO: 210 - protein, 11 aa, Homo sapiens
RASQSISIYLN

SEQ ID NO: 211 - protein, 7 aa, Homo sapiens
AASSLQS

SEQ ID NO: 212 - protein, 7 aa, Homo sapiens
AAASLQS

SEQ ID NO: 213 - protein, 9 aa, Homo sapiens
QQSYSSPIT

SEQ ID NO: 214 - protein, 9 aa, Homo sapiens
QQSYSAPIT

SEQ ID NO: 215 - protein, 10 aa, Homo sapiens
GFTFSSYAMN

SEQ ID NO: 216 - protein, 17 aa, Homo sapiens
TISGSGDNTYYADSVKG

SEQ ID NO: 217 - protein, 17 aa, Homo sapiens
TISGSGGNTYYADSVKG

SEQ ID NO: 218 - protein, 12 aa, Homo sapiens
KFVLMVYAMLDY

SEQ ID NO: 219 - protein, 11 aa, Homo sapiens
RASQRISNYLS

SEQ ID NO: 220 - protein, 16 aa, Homo sapiens
RSSQSLLHSNGYNFLN

SEQ ID NO: 221 - protein, 14 aa, Homo sapiens
TGTSSDVGNYNLVS

SEQ ID NO: 222 - protein, 14 aa, Homo sapiens
TGSSSNIGAGYDVH

SEQ ID NO: 223 - protein, 14 aa, Homo sapiens
TGSSSNIGAHYDVH

SEQ ID NO: 224 - protein, 13 aa, Homo sapiens
SGSNSNIGNNYVS

SEQ ID NO: 225 - protein, 11 aa, Homo sapiens
SGDKLGDKYAC

SEQ ID NO: 226 - protein, 12 aa, Homo sapiens
TLSSGYSSYEVD

SEQ ID NO: 227 - protein, 7 aa, Homo sapiens
LGSHRAS

SEQ ID NO: 228 - protein, 7 aa, Homo sapiens
EVSKRPS

SEQ ID NO: 229 - protein, 7 aa, Homo sapiens
GNSNRPS

SEQ ID NO: 230 - protein, 7 aa, Homo sapiens
GNTYRPS

SEQ ID NO: 231 - protein, 7 aa, Homo sapiens
SNNQRPS

SEQ ID NO: 232 - protein, 7 aa, Homo sapiens
DNNKRPS

SEQ ID NO: 233 - protein, 7 aa, Homo sapiens
QNTKWPL

SEQ ID NO: 234 - protein, 7 aa, Homo sapiens
VDTGGIV

SEQ ID NO: 235 - protein, 9 aa, Homo sapiens
QQSYSTPLI

SEQ ID NO: 236 - protein, 9 aa, Homo sapiens
MQVLQTPFT

SEQ ID NO: 237 - protein, 10 aa, Homo sapiens
CSYAGSSTLV

SEQ ID NO: 238 - protein, 11 aa, Homo sapiens
QSYDSSLSGSV

SEQ ID NO: 239 - protein, 11 aa, Homo sapiens
QSYDNSLSGVV

SEQ ID NO: 240 - protein, 11 aa, Homo sapiens
AVWDDSLNGWV

SEQ ID NO: 241 - protein, 11 aa, Homo sapiens
GTWDSSLSAVV

SEQ ID NO: 242 - protein, 9 aa, Homo sapiens
QAWDSSTVV

SEQ ID NO: 243 - protein, 18 aa, Homo sapiens
SDYHCGADHGSGTNFVVV

SEQ ID NO: 244 - protein, 10 aa, Homo sapiens
GYTFTSYGIS

SEQ ID NO: 245 - protein, 10 aa, Homo sapiens
GFTFSSYAMS

SEQ ID NO: 246 - protein, 10 aa, Homo sapiens
GFTFSSYGMH

SEQ ID NO: 247 - protein, 10 aa, Homo sapiens
GFTFSSYSMN

SEQ ID NO: 248 - protein, 12 aa, Homo sapiens
GGSISSGGYYWS

SEQ ID NO: 249 - protein, 12 aa, Homo sapiens
GGSISSSDYYWS

SEQ ID NO: 250 - protein, 10 aa, Homo sapiens
GGSFSAYYWN

SEQ ID NO: 251 - protein, 12 aa, Homo sapiens
GDSVSSNSAAWN

SEQ ID NO: 252 - protein, 17 aa, Homo sapiens
WISTYNGNTNYAQKVQG

SEQ ID NO: 253 - protein, 17 aa, Homo sapiens
TISGSGGRTYYADSVKG

SEQ ID NO: 254 - protein, 17 aa, Homo sapiens
VIWYDGSDKYYADSVKG

SEQ ID NO: 255 - protein, 17 aa, Homo sapiens
IIWYDGSNKYYADSVKG

SEQ ID NO: 256 - protein, 17 aa, Homo sapiens
SISSSSSYISYADSVKG

SEQ ID NO: 257 - protein, 16 aa, Homo sapiens
YIYNSGSTYYNPSLKS

SEQ ID NO: 258 - protein, 16 aa, Homo sapiens
YIYYSGSTYYNPSLKS

SEQ ID NO: 259 - protein, 16 aa, Homo sapiens
EINHSGRTDYNPSLKS

SEQ ID NO: 260 - protein, 18 aa, Homo sapiens
RTYYRSKWYKNYSVSVKS

SEQ ID NO: 261 - protein, 6 aa, Homo sapiens
GYTRDY

SEQ ID NO: 262 - protein, 8 aa, Homo sapiens
EVGSPFDY

SEQ ID NO: 263 - protein, 14 aa, Homo sapiens
ETGPLKLYYYGMDV

SEQ ID NO: 264 - protein, 13 aa, Homo sapiens
RGGLAARPGGMDV

SEQ ID NO: 265 - protein, 14 aa, Homo sapiens
DYDFWSAYYDAFDV

SEQ ID NO: 266 - protein, 11 aa, Homo sapiens
EDTAMVPYFDY

SEQ ID NO: 267 - protein, 12 aa, Homo sapiens
GGVTTYYYAMDV

SEQ ID NO: 268 - protein, 8 aa, Homo sapiens
GQLVPFDY

SEQ ID NO: 269 - protein, 9 aa, Homo sapiens
GGPTAAFDY

SEQ ID NO: 270 - protein, 109 aa, Homo sapiens
QSALTQPASVSGSPGQSITISCTGTSSDVGGYNSVSWYQQHPGKAPKLMIYEVSNRPSGVFNRFSGSKSGNTASLTISGLQAEDEADYYCNSYTSTSMVFGGGTKLTVL

SEQ ID NO: 271 - protein, 109 aa, Homo sapiens
QSALTQPASVFGSPGQSITISCTGTSSDVGAYNSVSWYQQHPGKAPKRMIYEVSNRPSGVSNRFSGSKSGNTASLTISGLQAEDEADYYCSSYTSTNMVFGGGTKLTVL

SEQ ID NO: 272 - protein, 109 aa, Homo sapiens; identical to SEQ ID NO: 31

SEQ ID NO: 273 - protein, 109 aa, Homo sapiens
QSVLTQPPSASGPPGQRVTIFCSGSSSNIGSNTVNWYQQLPGTAPKLLIYSNNRRPSGVPDRFSGSKSGTSASLAISGLQSEDEADYYCAAWDDSLNWVFGGGTKLTVL

SEQ ID NO: 274 - protein, 106 aa, Homo sapiens
SYELTQPPSVSVSPGQTASITCSGDKLGDKYACWYQQKPGQSPVLVIYQDSKRPSGIPERFSGSNSGNTATLTISGTQAMDEADYYCQAWDSSTVVFGGGTKLTVL

SEQ ID NO: 275 - protein, 106 aa, Homo sapiens; identical to SEQ ID NO: 44

SEQ ID NO: 276 - protein, 107 aa, Homo sapiens; identical to SEQ ID NO: 43

SEQ ID NO: 277 - protein, 107 aa, Homo sapiens
SYELIQPPSVSVSPGQTASITCSGDKLGDKYACWYQRKPGQSPILVIYQDTKRPSGIPERFSGSNSGNTATLTISGTQAMDEADYYCQAWDSSTAVVFGGGTKLTVL

SEQ ID NO: 278 - protein, 120 aa, Homo sapiens
QVQLQESGPGLVKPSETLSLTCTVSGGSISTYYWSWIRQPPGKGLEWIGYIYYSGSTNYNPSLKSRVTISVDTSKNQFSLKLSSVTAADTAVYYCARGSYSSGWFEFDYWGQGTLVTVSS

SEQ ID NO: 279 - protein, 12 aa, Homo sapiens
TLSSGYSSYEVD

SEQ ID NO: 280 - protein, 12 aa, Homo sapiens
VDTGGIVGSKGE

SEQ ID NO: 281 - protein, 13 aa, Homo sapiens
GADHGSGTNFVVV

SEQ ID NO: 282 - protein, 22 aa, Homo sapiens
QPVLTQPLFASASLGASVTLTC

SEQ ID NO: 283 - protein, 15 aa, Homo sapiens
WYQQRPGKGPRFVMR

SEQ ID NO: 284 - protein, 32 aa, Homo sapiens
GIPDRFSVLGSGLNRYLTIKNIQEEDESDYHC

SEQ ID NO: 285 - protein, 10 aa, Homo sapiens
FGGGTKLTVL

SEQ ID NO: 286 - protein, 108 aa, Homo sapiens
QSALTQPASVSGSPGQSITISCTGTSSDVGRYNSVSWYQHHPGKAPKVMIYEVSNRPSGVSTRFSGSKSGNTASLTISGLQAEDEADYYCSSYTSSSVVFGGGTKLTV

SEQ ID NO: 287 - protein, 108 aa, Homo sapiens
QSALTQPASVSGSPGQSITISCTGTSSDVGGYNSVSWYQQHPGKPPKLMIYEVSNRPSGVSIRFSGSKSGNTASLTISGLQAEDEADYFCSSYTSTSMVFGGGTKLTV

SEQ ID NO: 288 - protein, 108 aa, Homo sapiens
QSALTQPASVSGSPGQSITISCTGTNSDVGGYNSVSWYQQHPGKPPKLMIYEVSNRPSGISNRFSGSKSGNTASLTISGLQAEDEADYFCSSYTSTSMVFGGGTKLTV

SEQ ID NO: 289 - protein, 122 aa, Homo sapiens
QVHLVESGGGVVQPGRSLRLSCAASGFTFSSFGMHWVRQAPGKGLEWVALIWNDGSNKYYADSVKGRFTISRDNSKNTLYLQMNSLRAEDTAVYYCARAIAALYYYYGMDVWGHGTTVTVSS

SEQ ID NO: 290 - protein, 122 aa, Homo sapiens
QVQLVESGGGVVQPGRSLRLSCAASGFTFSSYGMHWVRQAPGKGLECVAIIWYDGSNKYYADSVKGRFTISRDNSKNTLYLQMNSLRAEDTAVYYCARRGGLAARPGGMDVWGQGTTVTVSS

SEQ ID NO: 291 - protein, 121 aa, Homo sapiens
QVQLVESGGGVVQPGRSLRLSCAASGFTFSSFGMHWVRQAPGKGLEWVALIWNDGSNKYYADSVKGRFTISRDNSKNTLYLQMNSLRAEDTAVYYCARAIAALYYYYGMDVWGQGTTVTVS

SEQ ID NO: 292 - protein, 119 aa, Homo sapiens
QVQLVESGGGVVQPGRSLRLSCAASGFTFSSYGMHWVRQAPGKGLEWVAIIWYDGSNKYYADSVKGRFTISRDNSKNTLYLQMNSLRAEDTAVYYCARRGGLPGGMDVWGQGTTVTVSS

SEQ ID NO: 293 - DNA, 327 bp, Homo sapiens
  source 1..327: mol_type = unassigned DNA
cagtctgccctgactcagcctgcctccgtgtctgggtctcctggacagtcgatcaccatctcctgcactggaaccagcagtgacgttggtggttataactctgtctcctggtaccaacagcacccaggcaaagcccccaaactcatgatttatgaggtcagtaatcggccctcaggggtttctaatcgcttctctggctccaagtctggcaacacggcctccctgaccatctctgggctccaggctgaggacgaggctgattattactgcaactcatatacaagcaccagcatggtattcggcggagggaccaagctgaccgtccta

SEQ ID NO: 294 - DNA, 327 bp, Homo sapiens
  source 1..327: mol_type = unassigned DNA
cagtctgccctgactcagcctgcctccgtgtctgggtctcctggacagtcgatcaccatctcctgcactggaaccagcagtgacgttggtggttataactctgtctcctggtaccaacagcacccaggcaaaccccccaaactcatgatttatgaggtcagtaatcggccctcaggggtttctaatcgcttctctggctccaagtctggcaacacggcctccctgaccatctctgggctccaggctgaggacgaggctgattatttctgcagctcatatacaagcaccagcatggtcttcggcggagggaccaagctgaccgtccta

SEQ ID NO: 295 - DNA, 318 bp, Homo sapiens
  source 1..318: mol_type = unassigned DNA
tcctatgagctgactcagccaccctcagtgtccgtgtccccaggacagacagccagaatcacctgctctggagataaattgggggataaatatgcttgctggtatcagcagaagccaggccagtcccctgtgctggtcatctatcaaaataccaagtggcccttagggatccctgagcgattctctggctccaagtctgggaacacagtcactctgaccatcagcgggacccaggctatggatgaggctgactattactgtcaggcgtgggacagcagcactgtggtattcggcggagggaccaagctgaccgtccta

SEQ ID NO: 296 - DNA, 327 bp, Homo sapiens; identical to SEQ ID NO: 95
  source 1..327: mol_type = unassigned DNA

SEQ ID NO: 297 - protein, 215 aa, Homo sapiens
ESALTQPASVSGSPGQSITISCTGTSSDVGGYNSVSWYQQHPGKAPKLMIYEVSNRPSGVSNRFSGSKSGNTASLTISGLQAEDEADYYCNSYTSTSMVFGGGTKLTVLGQPKAAPSVTLFPPSSEELQANKATLVCLISDFYPGAVTVAWKADSSPVKAGVETTTPSKQSNNKYAASSYLSLTPEQWKSHRSYSCQVTHEGSTVEKTVAPTECS

SEQ ID NO: 298 - protein, 230 aa, Homo sapiens
EVQLVQSGAEVKKPGASVKVSCKASGYTLTSYGISWVRQAPGQGLEWMGWVSFYNGNTNYAQKLQGRGTMTTDPSTSTAYMELRSLRSDDTAVYYCARGYGMDVWGQGTTVTVSSASTKGPSVFPLAPSSKSTSGGTAALGCLVKDYFPEPVTVSWNSGALTSGVHTFPAVLQSSGLYSLSSVVTVPSSSLGTQTYICNVNHKPSNTKVDKKVEPKSCAADEVDHHHHHH

SEQ ID NO: 299 - protein, 217 aa, Homo sapiens
ESVLTQPPSVSGAPGQRVTISCTGSSSNIGAGYDVHWYQQLPGTAPKLLISGNSNRPSGVPDRFSGSKSGTSASLAITGLQAEDEADYYCQSYDSSLSGSVFGGGTKLTVLGQPKAAPSVTLFPPSSEELQANKATLVCLISDFYPGAVTVAWKADSSPVKAGVETTTPSKQSNNKYAASSYLSLTPEQWKSHRSYSCQVTHEGSTVEKTVAPTECS

SEQ ID NO: 300 - protein, 238 aa, Homo sapiens
EVQLVESGGGLVKPGGSLRLSCAASGFTFSSYSMNWVRQAPGKGLEWVSSISSSSSYISYADSVKGRFTISRDNAKNSLYLQMNSLRAEDTAVYFCARDYDFWSAYYDAFDVWGQGTMVTVSSASTKGPSVFPLAPSSKSTSGGTAALGCLVKDYFPEPVTVSWNSGALTSGVHTFPAVLQSSGLYSLSSVVTVPSSSLGTQTYICNVNHKPSNTKVDKKVEPKSCAADEVDHHHHHH

SEQ ID NO: 301 - protein, 218 aa, Homo sapiens
ALQSVLTQPPSASGTPGQRVTISCSGSSSNIGSNTVNWYQQLPGTAPKLLIYSNNQRPSGVPDRFSGSKSGTSASLAISGLQSEDEADYYCAVWDDSLNGWVFGGGTKLTVLGQPKAAPSVTLFPPSSEELQANKATLVCLISDFYPGAVTVAWKADSSPVKAGVETTTPSKQSNNKYAASSYLSLTPEQWKSHRSYSCQVTHEGSTVEKTVAPTECS

SEQ ID NO: 302 - protein, 231 aa, Homo sapiens
QVQLQQWGAGLLKPSETLSLTCAVYGGSFSAYYWNWIRQPPGKGLEWIGEINHSGRTDYNPSLKSRVTISVDTSKKQFSLKLNSVTAADTAVYYCARGQLVPFDYWGQGTLVTVSSASTKGPSVFPLAPSSKSTSGGTAALGCLVKDYFPEPVTVSWNSGALTSGVHTFPAVLQSSGLYSHSSVVTVPSSSLGTQTYICNVNHKPSNTKVDKKVEPKSCAADEVDHHHHHH

SEQ ID NO: 303 - protein, 680 aa, Homo sapiens
QEDEDGDYEELVLALRSEEDGLAEAPEHGTTATFHRCAKDPWRLPGTYVVVLKEETHLSQSERTARRLQAQAARRGYLTKILHVFHGLLPGFLVKMSGDLLELALKLPHVDYIEEDSSVFAQSIPWNLERITPPRYRADEYQPPDGGSLVEVYLLDTSIQSDHREIEGRVMVTDFENVPEEDGTRFHRQASKCDSHGTHLAGVVSGRDAGVAKGASMRSLRVLNCQGKGTVSGTLIGLEFIRKSQLVQPVGPLVVLLPLAGGYSRVLNAACQRLARAGVVLVTAAGNFRDDACLYSPASAPEVITVGATNAQDQPVTLGTLGTNFGRCVDLFAPGEDIIGASSDCSTCFVSQSGTSQAAAHVAGIAAMMLSAEPELTLAELRQRLIHFSAKDVINEAWFPEDQRVLTPNLVAALPPSTHGAGWQLFCRTVWSAHSGPTRMATAIARCAPDEELLSCSSFSRSGKRRGERMEAQGGKLVCRAHNAFGGEGVYAIARCCLLPQANCSVHTAPPAEASMGTRVHCHQQGHVLTGCSSHWEVEDLGTHKPPVLRPRGQPNQCVGHREASIHASCCHAPGLECKVKEHGIPAPQEQVTVACEEGWTLTGCSALPGTSHVLGAYAVDNTCVVRSRDVSTTGSTSEEAVTAVAICCRSRHLAQASQELQGSSDYKDDDKHHHHHHHH

SEQ ID NO: 304 - protein, 680 aa, Homo sapiens
RRRRRRRRRRRRLRRRRRRRRRRRRRRHRRRRRFRRCRRRPWRRPGRYVVVLRRRRRRSRSRETAEELQRRAREEGRRTKIRRRFRGLLPGFLVRMRRRLRRLARRLPRVRYIEEDSSVFRQRIPRNRREIRPPRYRARRRRPPRGGRRVEVYLLDTRIRRRHEEIRGRVRRRRFRRRPRRRRREREERRRRCDRRGTHLAGVVSGERAGVARRARMRSLEVLNCRGRGRVSGTLIGLERIERRRRRRPRRPLVVLLPLAGRYSEVLNRACRRLAERGVVLVTAAGNFEDDACRYSPARAPEVITVGATNRRRRPVRRGRRGTNFGRCVDLFAPGRRIIGASSRCSRCRRRRSGTSQAAAHVAGIAARMLRRRPRLRRARLRQELRRRSRRRRIRRRRFPRRRERLTPRLVARLPPRRRRRGRRLFCRTVWSRRSGPRERARAIAECAPREELLSCSSFSRSGKRRGERMERQGGKLVCRAHNARRGRGVYAIARCCLLPQARCSVHRAPPARRRRGTEVRCRRRGHVLTGCSSHWRRRDRGTRKPPRLRPEGRPRQCVGHREASIHASCCHAPGLECRRRRRRIPAPRERVTVRCRRGWTLTGCSALPGTSHVLGAYARDNTCVVRSEDRRRRRRRRRERVTAVAICCESEHLAQASQELQGSSDYKDDDKHHHHHHHH

SEQ ID NO: 305 - protein, 14 aa, Homo sapiens
TGTSSDVGGYNSVS

SEQ ID NO: 306 - protein, 7 aa, Homo sapiens
EVSNRPS

SEQ ID NO: 307 - protein, 9 aa, Homo sapiens
SSYTSTSMV

SEQ ID NO: 308 - protein, 5 aa, Homo sapiens
SYGIS

SEQ ID NO: 309 - protein, 17 aa, Homo sapiens
WISAYNGNTNYAQKVQG

SEQ ID NO: 310 - protein, 6 aa, Homo sapiens
GYGMDV

SEQ ID NO: 311 - protein, 14 aa, Homo sapiens
TGTSSDVGRYNSVS

SEQ ID NO: 312 - protein, 7 aa, Homo sapiens
EVSNRPS

SEQ ID NO: 313 - protein, 9 aa, Homo sapiens
SSYTSSSVV

SEQ ID NO: 314 - protein, 17 aa, Homo sapiens
WISAYNGNTNYAEKLQG

SEQ ID NO: 315 - protein, 6 aa, Homo sapiens
GYVMDV

SEQ ID NO: 316 - protein, 14 aa, Homo sapiens
TGTSSDVGAYNSVS

SEQ ID NO: 317 - protein, 9 aa, Homo sapiens
SSYTSTNMV

SEQ ID NO: 318 - protein, 17 aa, Homo sapiens
WVSAYNGNTNYAQKFQG

SEQ ID NO: 319 - protein, 9 aa, Homo sapiens
NSYTSTSMV

SEQ ID NO: 320 - protein, 17 aa, Homo sapiens
WVSFYNGNTNYAQKLQG

SEQ ID NO: 321 - protein, 7 aa, Homo sapiens
EVTNRPS

SEQ ID NO: 322 - protein, 14 aa, Homo sapiens
TGTNSDVGGYNSVS

SEQ ID NO: 323 - protein, 17 aa, Homo sapiens
WISVYNGNTNYAQKVQG

SEQ ID NO: 324 - protein, 17 aa, Homo sapiens
WISFYNGNTNYAQKVQG

SEQ ID NO: 325 - protein, 13 aa, Homo sapiens
SGSSSNIGNNFVS

SEQ ID NO: 326 - protein, 7 aa, Homo sapiens
DYNKRPS

SEQ ID NO: 327 - protein, 11 aa, Homo sapiens
GTWDSSLSGYV

SEQ ID NO: 328 - protein, 5 aa, Homo sapiens
SFGMH

SEQ ID NO: 329 - protein, 17 aa, Homo sapiens
LIWNDGSNKYYADSVKG

SEQ ID NO: 330 - protein, 13 aa, Homo sapiens
AIAALYYYYGMDV

SEQ ID NO: 331 - protein, 7 aa, Homo sapiens
DSNKRPS

SEQ ID NO: 332 - protein, 11 aa, Homo sapiens
GTWDSSLSAYV

SEQ ID NO: 333 - protein, 5 aa, Homo sapiens
SYGMH

SEQ ID NO: 334 - protein, 17 aa, Homo sapiens
LIWHDGSNTYYVDSVKG

SEQ ID NO: 335 - protein, 13 aa, Homo sapiens
GIAVAYYYYGMDV

SEQ ID NO: 336 - protein, 17 aa, Homo sapiens
LIWSDGSDEYYADSVKG

SEQ ID NO: 337 - protein, 11 aa, Homo sapiens
GTWDSSLSSYV

SEQ ID NO: 338 - protein, 17 aa, Homo sapiens
LIWSDGSDKYYADSVKG

SEQ ID NO: 339 - protein, 13 aa, Homo sapiens
SGSSSNIGSKTVN

SEQ ID NO: 340 - protein, 7 aa, Homo sapiens
SNNRRPS

SEQ ID NO: 341 - protein, 10 aa, Homo sapiens
AAWDDSLNWV

SEQ ID NO: 342 - protein, 4 aa, Homo sapiens
YWMS

SEQ ID NO: 343 - protein, 17 aa, Homo sapiens
NIKQDGSEKYYVDSVKG

SEQ ID NO: 344 - protein, 10 aa, Homo sapiens
ESNWGFAFDI

SEQ ID NO: 345 - protein, 13 aa, Homo sapiens
SGSSSNIGSNTVN

SEQ ID NO: 346 - protein, 5 aa, Homo sapiens
RYWMS

SEQ ID NO: 347 - protein, 17 aa, Homo sapiens
NIKHDGSEKYYVDSVKG

SEQ ID NO: 348 - protein, 10 aa, Homo sapiens
ESNWGFAFDV

SEQ ID NO: 349 - protein, 7 aa, Homo sapiens
RNNQRPL

SEQ ID NO: 350 - protein, 5 aa, Homo sapiens
SYWMS

SEQ ID NO: 351 - protein, 5 aa, Homo sapiens
NFWMS

SEQ ID NO: 352 - protein, 10 aa, Homo sapiens
RASQSISYLN

SEQ ID NO: 353 - protein, 6 aa, Homo sapiens
AASLQS

SEQ ID NO: 354 - protein, 8 aa, Homo sapiens
QQSYSPIT

SEQ ID NO: 355 - protein, 11 aa, Homo sapiens
RASQSISIYLN

SEQ ID NO: 356 - protein, 7 aa, Homo sapiens
AAASLQS

SEQ ID NO: 357 - protein, 9 aa, Homo sapiens
QQSYSAPIT

SEQ ID NO: 358 - protein, 11 aa, Homo sapiens
RASQSISSYLN

SEQ ID NO: 359 - protein, 7 aa, Homo sapiens
AASSLQS

SEQ ID NO: 360 - protein, 9 aa, Homo sapiens
QQSYSSPIT

SEQ ID NO: 361 - protein, 5 aa, Homo sapiens
SYAMN

SEQ ID NO: 362 - protein, 16 aa, Homo sapiens
TISGSGNTYYADSVKG

SEQ ID NO: 363 - protein, 12 aa, Homo sapiens
KFVLMVYAMLDY

SEQ ID NO: 364 - protein, 17 aa, Homo sapiens
TISGSGGNTYYADSVKG

SEQ ID NO: 365 - protein, 17 aa, Homo sapiens
TISGSGDNTYYADSVKG

SEQ ID NO: 366 - protein, 10 aa, Homo sapiens
GYSLTSYGIS

SEQ ID NO: 367 - protein, 10 aa, Homo sapiens
GYALTSYGIS

SEQ ID NO: 368 - protein, 10 aa, Homo sapiens
GYTLTSYGIS

SEQ ID NO: 369 - protein, 10 aa, Homo sapiens
GYSFTSYGIS

SEQ ID NO: 370 - protein, 10 aa, Homo sapiens
GYTFPSYGIS

SEQ ID NO: 371 - protein, 10 aa, Homo sapiens
GFTFSSYWMS

SEQ ID NO: 372 - protein, 10 aa, Homo sapiens
GFTFSRYWMS

SEQ ID NO: 373 - protein, 10 aa, Homo sapiens
GLTFSNFWMS

SEQ ID NO: 374 - protein, 10 aa, Homo sapiens
GFTFSSYAMN

SEQ ID NO: 375 - protein, 10 aa, Homo sapiens
GFTFNSFGMH

SEQ ID NO: 376 - protein, 10 aa, Homo sapiens
GFTFRSYGMH

SEQ ID NO: 377 - protein, 16 aa, Homo sapiens
NIKQDGSEKYVDSVKG

SEQ ID NO: 378 - protein, 16 aa, Homo sapiens
NIKHDGSEKYVDSVKG

SEQ ID NO: 379 - protein, 16 aa, Homo sapiens
TISGSGDNTYADSVKG

SEQ ID NO: 380 - protein, 16 aa, Homo sapiens
TISGSGGNTYADSVKG

SEQ ID NO: 381 - protein, 16 aa, Homo sapiens
LIWNDGSNKYADSVKG

SEQ ID NO: 382 - protein, 16 aa, Homo sapiens
LIWSDGSDEYADSVKG

SEQ ID NO: 383 - protein, 16 aa, Homo sapiens
LIWSDGSDKYADSVKG

SEQ ID NO: 384 - protein, 16 aa, Homo sapiens
LIWHDGSNTYVDSVKG

SEQ ID NO: 385 - protein, 10 aa, Homo sapiens
ESNWGFAFDI

SEQ ID NO: 386 - protein, 10 aa, Homo sapiens
ESNWGFAFDV

SEQ ID NO: 387 - protein, 6 aa, Homo sapiens
GYVMDV

SEQ ID NO: 388 - protein, 11 aa, Homo sapiens
RASQSISIYLN

SEQ ID NO: 389 - protein, 14 aa, Homo sapiens
TGTNSDVGGYNSVS

SEQ ID NO: 390 - protein, 14 aa, Homo sapiens
TGTSSDVGAYNSVS

SEQ ID NO: 391 - protein, 14 aa, Homo sapiens
TGTSSDVGRYNSVS

SEQ ID NO: 392 - protein, 7 aa, Homo sapiens
RNNQRPL

SEQ ID NO: 393 - protein, 7 aa, Homo sapiens
AAASLQS

SEQ ID NO: 394 - protein, 9 aa, Homo sapiens
QQSYSAPIT

SEQ ID NO: 395 - protein, 9 aa, Homo sapiens
NSYTSTSMV

SEQ ID NO: 396 - protein, 9 aa, Homo sapiens
SSYTSSSVV

SEQ ID NO: 397 - protein, 10 aa, Homo sapiens
AAWDDSLNWV

SEQ ID NO: 398 - protein, 11 aa, Homo sapiens
GTWDSSLSSYV

SEQ ID NO: 399 - protein, 11 aa, Homo sapiens
GTWDSSLSAYV

SEQ ID NO: 400 - protein, 116 aa, Homo sapiens
QVQLQESGPGLVKPSETLSLTCTVSGGSISSYYWSWIRQPPGKGLEWIGYIYYSGSTNYNPSLKSRVTISVDTSKNQFSLKLSSVTAADTAVYYCARYSSGWFDYWGQGTLVTVSS

SEQ ID NO: 401 - protein, 118 aa, Homo sapiens
EVQLVESGGGLVQPGGSLRLSCVVSGFTFSSYWMSWVRQAPGKGLEWVANIKQDGSEKYYVDSVKGRFTISRDNAKNSLYLQMNSLRAEDTAVYYCARESNWGFAFDIWGQGTMVTVS

SEQ ID NO: 402 - protein, 115 aa, Homo sapiens
EVQLVESGGGLVQPGGSLRLSCAASGFTFSSYWMSWVRQAPGKGLEWVANIKQDGSEKYYVDSVKGRFTISRDNAKNSLYLQMNSLRAEDTAVYYCARNWGAFDIWGQGTMVTVS

SEQ ID NO: 403 - protein, 6 aa, Homo sapiens
ENLYFQ

SEQ ID NO: 404-417 - skipped (14 entries)

SEQ ID NO: 418 - DNA, 363 bp, Homo sapiens
  source 1..363: mol_type = unassigned DNA
caggtgcaggtggtgcagtctggggctgaggtgaagaagcctggggcctcagtgaaggtctcctgcaaggcttctggatacaccttcaccggctactatatacactgggtgcgacaggcccctggacaagggcttgagtggatgggatggatcaaccctcacagtggtggcgcaaactatgcacagaagtttcagggcagggtcaccatgaccagggacacgtccatcagcacagcctacatggagctgagcaggctgagatctgacgacacggccgtgtattactgtgcgagaggcaactggaactacgactactacggtatggacgtctggggccaagggaccacggtcaccgtctcctca

SEQ ID NO: 419 - protein, 121 aa, Homo sapiens
QVQVVQSGAEVKKPGASVKVSCKASGYTFTGYYIHWVRQAPGQGLEWMGWINPHSGGANYAQKFQGRVTMTRDTSISTAYMELSRLRSDDTAVYYCARGNWNYDYYGMDVWGQGTTVTVSS

SEQ ID NO: 420 - DNA, 321 bp, Homo sapiens
  source 1..321: mol_type = unassigned DNA
gacatccagatgacccagtctccatcctccctgtctgcatctgtaggagacagagtcaccatcacttgccgggcgagtcaggacattagcaattatttagcctggtatcagcagaaaccagggaaagttcctaagctcctgatctatgctgcatccactttgcaatcaggggtcccatctcggttcagtggcagtggatctgggacagatttcactctcaccatcagcagcctacagcctgaagatgttgcaacttatttctgtcaaaggtatcagattgccccattcactttcggccctgggaccaaggtggatatcaaa

SEQ ID NO: 421 - protein, 107 aa, Homo sapiens
DIQMTQSPSSLSASVGDRVTITCRASQDISNYLAWYQQKPGKVPKLLIYAASTLQSGVPSRFSGSGSGTDFTLTISSLQPEDVATYFCQRYQIAPFTFGPGTKVDIK

SEQ ID NO: 422 - DNA, 366 bp, Homo sapiens
  source 1..366: mol_type = unassigned DNA
caggtgcagctggtggagtctgggggaggcgtggtccagcctgggaggtccctgagactctcctgtgcagcgtctggattcaccttcagtagctatggcatgcactgggtccgccaggctccaggcaaggggctggagtgggtggcagttatctggtatgatggaagtactaaatactatgcagactccgtgaagggccgatccaccatctccagagacaattccaagaacacgctgtatctgcaaatgaacagcctgagagccgaggacacggctgtgtattactgtgcgaggtcagtggctggttaccactactactacggtatggacgtctggggccaagggaccacggtcaccgtctcctca

SEQ ID NO: 423 - protein, 122 aa, Homo sapiens
QVQLVESGGGVVQPGRSLRLSCAASGFTFSSYGMHWVRQAPGKGLEWVAVIWYDGSTKYYADSVKGRSTISRDNSKNTLYLQMNSLRAEDTAVYYCARSVAGYHYYYGMDVWGQGTTVTVSS

SEQ ID NO: 424 - DNA, 324 bp, Homo sapiens
  source 1..324: mol_type = unassigned DNA
tcttctgagctgactcaggaccctgctgtgtctgtggccttgggacagacagtcaggatcacatgccaaggagacagcctcagaggctattatgcaacctggtaccagcagaagccaagacaggcccctgtacttgtcatctatggtaaaaactaccggccctcagggatcccagaccgattctctggctccacctcaggaaacacagcttccttgaccatcactggggctcaggcggaagatgaggctgactattactgtaactcccgggacagcattggtaaccatctggtgttcggcggagggaccaagctgaccgtccta

SEQ ID NO: 425 - protein, 108 aa, Homo sapiens
SSELTQDPAVSVALGQTVRITCQGDSLRGYYATWYQQKPRQAPVLVIYGKNYRPSGIPDRFSGSTSGNTASLTITGAQAEDEADYYCNSRDSIGNHLVFGGGTKLTVL

SEQ ID NO: 426 - DNA, 366 bp, Homo sapiens
  source 1..366: mol_type = unassigned DNA
caggtgcagctggtggagtctgggggaggcgtggtccagcctgggaggtccctgagactctcctgtgcagcgtctggattcaccttcagtagctatggcttgcactgggtccgccaggctccaggcaaggggctggagtgggtggcagttatatggttagatggaagtaataaatactatgcagactccgtgaagggccgatccaccatctccagagacaattccaagaacacgctgtatctgcaaatgaacagcctgagagccgaggacacggctgtgtattactgtgcgaggtcagtggctggttaccactactactacggtatggacgtctggggccaagggaccacggtcaccgtctcctca

SEQ ID NO: 427 - protein, 122 aa, Homo sapiens
QVQLVESGGGVVQPGRSLRLSCAASGFTFSSYGLHWVRQAPGKGLEWVAVIWLDGSNKYYADSVKGRSTISRDNSKNTLYLQMNSLRAEDTAVYYCARSVAGYHYYYGMDVWGQGTTVTVSS

SEQ ID NO: 428 - DNA, 324 bp, Homo sapiens
  source 1..324: mol_type = unassigned DNA
tcttctgagctgactcaggaccctgctgtgtctgtggccttgggacagacagtcaggatcacatgccaaggagacagcctcagaagttattatggaagctggtaccagcagaagccaagacaggcccctgtacttgtcatctttggtaaaaacaaccggccctcagggatcccagaccgattctctggctccacctcaggaaacacagcttccttgaccatcactggggctcaggcggaagatgaggctgactattactgtaactcacgggacatcattggtgaccatctgctgttcggcggagggaccaagctgaccgtccta

SEQ ID NO: 429 - protein, 108 aa, Homo sapiens
SSELTQDPAVSVALGQTVRITCQGDSLRSYYGSWYQQKPRQAPVLVIFGKNNRPSGIPDRFSGSTSGNTASLTITGAQAEDEADYYCNSRDIIGDHLLFGGGTKLTVL

SEQ ID NO: 430 - DNA, 366 bp, Homo sapiens
  source 1..366: mol_type = unassigned DNA
caggtgcagctggtggagtctgggggaggcgtggtccagtctgggaggtccctgagactctcctgtgcagcgtctggattcaccttcaggaactatggcatgcactgggtccgccaggctccaggcaaggggctggagtgggtggcagttatatggtttgatggaagtaataaatactatgcagactccgtgaagggccgatccaccatctccagagacaattccaagaacacgctgtatctgctaatgaacagcctgagagccgaggacacggctgtgtattactgtgcgaggtcagtggctggttaccactactactacggtatggacgtctggggccaagggaccacggtcaccgtctcctca

SEQ ID NO: 431 - protein, 122 aa, Homo sapiens
QVQLVESGGGVVQSGRSLRLSCAASGFTFRNYGMHWVRQAPGKGLEWVAVIWFDGSNKYYADSVKGRSTISRDNSKNTLYLLMNSLRAEDTAVYYCARSVAGYHYYYGMDVWGQGTTVTVSS

SEQ ID NO: 432 - DNA, 324 bp, Homo sapiens
  source 1..324: mol_type = unassigned DNA
tcttctgagctgactcaggaccctgctgtgtctgtggccttgggacagacagtcaggatcacatgccagggagacagcctcagaagctattatgcaagctggtaccagcagaagccaagacaggcccctgtacttgtcatctatggtaaaaacaaccggccctcagggatcccagaccgaatctctggctccacctcaggaaacacagcttccttgaccatcactggggctcaggcggaagatgaggctgactattactgtaaatcccgggacatcattggtgaccatctggtgttcggcggagggaccaaactgaccgtccta

SEQ ID NO: 433 - protein, 108 aa, Homo sapiens
SSELTQDPAVSVALGQTVRITCQGDSLRSYYASWYQQKPRQAPVLVIYGKNNRPSGIPDRISGSTSGNTASLTITGAQAEDEADYYCKSRDIIGDHLVFGGGTKLTVL

SEQ ID NO: 434 - DNA, 342 bp, Homo sapiens
  source 1..342: mol_type = unassigned DNA
caggtgcagctggtggagtctgggggaggcgtggtccagcctgggaggtccctgagactctcctgtgcagcgtctggattcaccttcagtagctatggcatgcactgggtccgccaggctccaggcaaggggctggagtgggtggcagttatatggtatgatggaagtaataaatactatgcagactccgtgaagggccgattcaccatctccagagacaattccaagaacacgctgtatctgcaaatgaacagcctgagagccgaggacacggctgtgtattactgtgtgagagatcggggactggactggggccagggaaccctggtcaccgtctcctca

SEQ ID NO: 435 - protein, 114 aa, Homo sapiens
QVQLVESGGGVVQPGRSLRLSCAASGFTFSSYGMHWVRQAPGKGLEWVAVIWYDGSNKYYADSVKGRFTISRDNSKNTLYLQMNSLRAEDTAVYYCVRDRGLDWGQGTLVTVSS

SEQ ID NO: 436 - DNA, 324 bp, Homo sapiens
  source 1..324: mol_type = unassigned DNA
tcttctgagctgactcaggaccctgctgtgtctgtggccttgggacagacagtcaggatcacatgccaaggagacagcctcagaggctattatgcaagctggtaccagcagaagccaagacaggcccctgtacttgtcatctatggtaaaaacaaccggccctcagggatcccagaccgattctctggctccacctcaggaaacacagcttccttgaccatcactggggctcaggcggaagatgaggctgactattactgtaagtcccgggacagcagtggtgaccatctggtgttcggcggagggaccaagctgaccgtccta

SEQ ID NO: 437 - protein, 108 aa, Homo sapiens
SSELTQDPAVSVALGQTVRITCQGDSLRGYYASWYQQKPRQAPVLVIYGKNNRPSGIPDRFSGSTSGNTASLTITGAQAEDEADYYCKSRDSSGDHLVFGGGTKLTVL

SEQ ID NO: 438 - DNA, 366 bp, Homo sapiens
  source 1..366: mol_type = unassigned DNA
caggtgcaggtggtggagtctgggggaggcgtggtccagcctggggggtccctgagactctcctgtgcagcgtctggattcaccttcagtaactatggcatgcactgggtccgccaggctccaggcaaggggctggagtgggtggcagttatttggtatgatggaagtagtaaatactatgcagactccgtgaagggccgatccaccatctccagagacaattccaagaacacggtgtatctgcaaatgaacagcctgagagccgaggacacggctgtgtattactgtgcgaggtcagtggctggttaccactactactacggtatggacgtctggggccaagggaccacggtcaccgtctcctca

SEQ ID NO: 439 - protein, 122 aa, Homo sapiens
QVQVVESGGGVVQPGGSLRLSCAASGFTFSNYGMHWVRQAPGKGLEWVAVIWYDGSSKYYADSVKGRSTISRDNSKNTVYLQMNSLRAEDTAVYYCARSVAGYHYYYGMDVWGQGTTVTVSS

SEQ ID NO: 440 - DNA, 324 bp, Homo sapiens; identical to SEQ ID NO: 436
  source 1..324: mol_type = unassigned DNA

SEQ ID NO: 441 - protein, 108 aa, Homo sapiens; identical to SEQ ID NO: 437

SEQ ID NO: 442 - DNA, 366 bp, Homo sapiens
  source 1..366: mol_type = unassigned DNA
caggtgcagctggtggagtctgggggaggcgtggtccagcctgggaggtccctgagtctctcctgtgcagcgtctggattcaccttcagtagctatggcatgcactgggtccgccaggctccaggcaaggggctggagtgggtggcagttatatggtatgatggaagttataaagactatgcagactccgtgaagggccgatccaccatctccagagacaactccaagaacacgctgtatctgcaaatgaacagcctgagagccgaggacacggctgtgtattattgtgcgaggtcagtggctggttaccactactactacggtatggacgtctggggccaagggaccacggtcaccgtctcctca

SEQ ID NO: 443 - protein, 122 aa, Homo sapiens
QVQLVESGGGVVQPGRSLSLSCAASGFTFSSYGMHWVRQAPGKGLEWVAVIWYDGSYKDYADSVKGRSTISRDNSKNTLYLQMNSLRAEDTAVYYCARSVAGYHYYYGMDVWGQGTTVTVSS

SEQ ID NO: 444 - DNA, 324 bp, Homo sapiens
  source 1..324: mol_type = unassigned DNA
tcttctgagctgactcaggaccctgctgtgtctgtggccttgggacagacagtcaggatcacatgccaaggagacagcctcagaacctattatgcaagctggtaccagcagaagccaagacaggcccctattcttgtcatctatggtaaaaacaaccggccctcagggatcccagaccgattctctggctccacctcaggaatcacagcttccttgaccatcactggggctcaggcggaagatgaggctgactattactgtaaatcccgggacatcattggtaaccatctgctgttcggcggagggactaagctgaccgtccta

SEQ ID NO: 445 - protein, 108 aa, Homo sapiens
SSELTQDPAVSVALGQTVRITCQGDSLRTYYASWYQQKPRQAPILVIYGKNNRPSGIPDRFSGSTSGITASLTITGAQAEDEADYYCKSRDIIGNHLLFGGGTKLTVL

SEQ ID NO: 446 - DNA, 375 bp, Homo sapiens
  source 1..375: mol_type = unassigned DNA
caggtgcagctggtggcgtctgggggaggcgtggtccagcctgggaggtccctgagactctcctgtgcagcgtctggattcaccctcagtagctatggcatgcactgggtccgccaggctccaggccaggggctggagtgggtggcagtcatatggtatgatggaagtaacaaatactatgcagcctccgtgaagggccgattcaccatctccagagacaattccaagaacacgctgtatctgcaaatgaacagtctgagagccgaggacacggctgtgtattactgtgcgagagggggtggttcggggagtcatcgctactactactacggtatggacgtctggggccaagggaccacggtcaccgtctcctca

SEQ ID NO: 447 - protein, 125 aa, Homo sapiens
QVQLVASGGGVVQPGRSLRLSCAASGFTLSSYGMHWVRQAPGQGLEWVAVIWYDGSNKYYAASVKGRFTISRDNSKNTLYLQMNSLRAEDTAVYYCARGGGSGSHRYYYYGMDVWGQGTTVTVSS

SEQ ID NO: 448 - DNA, 324 bp, Homo sapiens; identical to SEQ ID NO: 444
  source 1..324: mol_type = unassigned DNA

SEQ ID NO: 449 - protein, 108 aa, Homo sapiens; identical to SEQ ID NO: 445

SEQ ID NO: 450 - DNA, 366 bp, Homo sapiens
  source 1..366: mol_type = unassigned DNA
caggtgcaagtggtggagtctgggggaggcgtggtccagcctgggaggtccctgagactctcctgtgcagcgtctggattcaccttcagtaactatggcatgcactgggtccgccaggctccaggcaaggggctggagtgggtggcagttatatggtatgatggaggtaataaatactatgcagactccgtgaagggccgatccatcatctccagagacaattccaagagcacgctgtatctgcaaatgaacagcctgagagccgaggacacggctgtttattattgtgcgaggtcagtggctggttaccattattactacggtatggacgtctggggccaagggaccacggtcaccgtcgcctca

SEQ ID NO: 451 - protein, 122 aa, Homo sapiens
QVQVVESGGGVVQPGRSLRLSCAASGFTFSNYGMHWVRQAPGKGLEWVAVIWYDGGNKYYADSVKGRSIISRDNSKSTLYLQMNSLRAEDTAVYYCARSVAGYHYYYGMDVWGQGTTVTVAS

SEQ ID NO: 452 - DNA, 327 bp, Homo sapiens
  source 1..327: mol_type = unassigned DNA
cagtctgccctgactcagcctgcctccgtgtctgggtctcctggacagtcgatcaccatctcctgcactggaaccagcagtgacgttggtggttataactctgtctcctggtaccaacagcacccaggcaaaccccccaaactcatgatttatgaggtcagtaatcggccctcagggatttctaatcgcttctctggctccaagtctggcaacacggcctccctgaccatctctgggctccaggctgaggacgaggctgattatttctgcagctcatatacaagcaccagcatggtcttcggcggagggaccaagctggccgtccta

SEQ ID NO: 453 - protein, 109 aa, Homo sapiens
QSALTQPASVSGSPGQSITISCTGTSSDVGGYNSVSWYQQHPGKPPKLMIYEVSNRPSGISNRFSGSKSGNTASLTISGLQAEDEADYFCSSYTSTSMVFGGGTKLAVL

SEQ ID NO: 454 - DNA, 366 bp, Homo sapiens; identical to SEQ ID NO: 450
  source 1..366: mol_type = unassigned DNA

SEQ ID NO: 455 - protein, 122 aa, Homo sapiens; identical to SEQ ID NO: 451

SEQ ID NO: 456 - DNA, 324 bp, Homo sapiens
  source 1..324: mol_type = unassigned DNA
tcttctgagctgactcaggaccctgctgtgtctgtggccttgggacagacagtcaggatcacatgccaaggagacagcctcagaggctattatgcaagctggtaccagcagaagccaagacaggcccctgtacttgtcatctatggtaaaaacaaccggccctcagggatcccagaccgattctctggctccacgtcaggaaacacagcttccttgaccatcactggggctcaggcggaagatgaggctgactattactgtaactcccgggacaacattggtgaccatctggtgttcggcggagggaccaagctgaccgtccta

SEQ ID NO: 457 - protein, 108 aa, Homo sapiens
SSELTQDPAVSVALGQTVRITCQGDSLRGYYASWYQQKPRQAPVLVIYGKNNRPSGIPDRFSGSTSGNTASLTITGAQAEDEADYYCNSRDNIGDHLVFGGGTKLTVL

SEQ ID NO: 458 - DNA, 381 bp, Homo sapiens
  source 1..381: mol_type = unassigned DNA
gaggtgcagctggtggagtctgggggaggcttggtccagcctggggggtccctgagactctcctgtgcagcctccggattcacctttagtagctattggatgagctgggtccgccaggctccagggaaggggctggagtgggtggccagcataaaacaagatggaagtgagaaatactatgtggactctgtgaagggccgattcaccatctccagagacaacgccaggaactcactgtatctgcaaatgaacagcctgagagccgaggacacggctgtgtattactgtgcgagagatcttgtattaatggtgtatgatatagactactactactacggtatggacgtctggggccaagggaccacggtcaccgtctcctca

SEQ ID NO: 459 - protein, 127 aa, Homo sapiens
EVQLVESGGGLVQPGGSLRLSCAASGFTFSSYWMSWVRQAPGKGLEWVASIKQDGSEKYYVDSVKGRFTISRDNARNSLYLQMNSLRAEDTAVYYCARDLVLMVYDIDYYYYGMDVWGQGTTVTVSS

SEQ ID NO: 460 - DNA, 336 bp, Homo sapiens
  source 1..336: mol_type = unassigned DNA
gatattgtgatgactcagtctccactctccctgcccgtcacccctggagagccggcctccatctcctgcaggtctagtcagagcctcctgcatagtaatggatacaactatttggattggtacctgcagaagccagggcagtctccacagctcctgatctatttgggttctaatcgggcctccggggtccctgacaggttcagtggcagtggatcaggcacagattttacactgaaaatcagcagagtggaggctgaggatgttggggtttattactgcatgcaagctctacaaactccgctcactttcggcggagggaccaaggtagagatcaaa

SEQ ID NO: 461 - protein, 112 aa, Homo sapiens
DIVMTQSPLSLPVTPGEPASISCRSSQSLLHSNGYNYLDWYLQKPGQSPQLLIYLGSNRASGVPDRFSGSGSGTDFTLKISRVEAEDVGVYYCMQALQTPLTFGGGTKVEIK

SEQ ID NO: 462 - DNA, 381 bp, Homo sapiens
  source 1..381: mol_type = unassigned DNA
gaggtgcagctggtggagtctgggggaggcttggtccagcctggggggtccctgagactctcctgtgcagcctccggattcacctttagtaactattggatgagctgggtccgccaggctccagggaaggggctggagtgggtggccagcataaaacaagatggaagtgagaaatactatgtggactctgtgaagggccgattcgccatctccagagacaacgccaagaactcactgtttctgcaaatgaacagcctgagagccgaggacacggctgtgtattactgtgcgagagatcttgtactaatggtgtatgatatagactactactactacggtatggacgtctggggccaagggaccacggtcaccgtctcctca

SEQ ID NO: 463 - protein, 127 aa, Homo sapiens
EVQLVESGGGLVQPGGSLRLSCAASGFTFSNYWMSWVRQAPGKGLEWVASIKQDGSEKYYVDSVKGRFAISRDNAKNSLFLQMNSLRAEDTAVYYCARDLVLMVYDIDYYYYGMDVWGQGTTVTVSS

SEQ ID NO: 464 - DNA, 336 bp, Homo sapiens
  source 1..336: mol_type = unassigned DNA
gatattgtgatgactcagtctccactctccctgcctgtcacccctggagagccggcctccatctcttgcaggtctagtcagagcctcctgcatagtaatgggtacaactatttggattggtacctgcagaagccagggcagtctccacagctcctgatctatttgggttctaatcgggcctccggggtccctgacaggttcagtggcagtggatcaggcacacatcttacactgaaaatcagcagagtggaggctgaggatgttggagtttattactgcatgcaaactctacaaactccgctcactttcggcggagggaccaaggtggagatcaaa

SEQ ID NO: 465 - protein, 112 aa, Homo sapiens
DIVMTQSPLSLPVTPGEPASISCRSSQSLLHSNGYNYLDWYLQKPGQSPQLLIYLGSNRASGVPDRFSGSGSGTHLTLKISRVEAEDVGVYYCMQTLQTPLTFGGGTKVEIK

SEQ ID NO: 466 - DNA, 342 bp, Homo sapiens
  source 1..342: mol_type = unassigned DNA
caggtgcagctggtggagtctgggggaggcgtggcccagcctgggaggtccctgagactctcctgtgcagcgtctggattcaccttcagtagctatggcatgcactgggtccgccaggctccaggcaaggggctggagtgggtggcagttatatactatgatggaattaataaacactatgcagactccgtgaagggccgattcaccatctccagagacaattccaagaacacgctgtatctgcaaatgaacagcctgagagccgaggacacggctgtgtattactgtgcgagagatcggggactggactggggccagggaaccctggtcaccgtctcctca

SEQ ID NO: 467 - protein, 114 aa, Homo sapiens
QVQLVESGGGVAQPGRSLRLSCAASGFTFSSYGMHWVRQAPGKGLEWVAVIYYDGINKHYADSVKGRFTISRDNSKNTLYLQMNSLRAEDTAVYYCARDRGLDWGQGTLVTVSS

SEQ ID NO: 468 - DNA, 339 bp, Homo sapiens
  source 1..339: mol_type = unassigned DNA
gacatcgtgatgacccagtctccagactccctggctgtgtctctgggcgagagggccaccatcaactgcaagtccagccagagtgttttatacagctccaacagtaagaactacttagtttggtaccagcagaaaccaggacagcctcctaagctgctcatttactgggcctctacccgggaatccggggtccctgaccgattcagtggcagcgggtctgggacagatttcactctcaccatcagcagcctgcaggctgaagatgtggcagtttattactgtcaacaatattatagtactccgtggacgttcggccaagggaccaaggtggaaatcaaa

SEQ ID NO: 469 - protein, 113 aa, Homo sapiens
DIVMTQSPDSLAVSLGERATINCKSSQSVLYSSNSKNYLVWYQQKPGQPPKLLIYWASTRESGVPDRFSGSGSGTDFTLTISSLQAEDVAVYYCQQYYSTPWTFGQGTKVEIK

SEQ ID NO: 470 - DNA, 357 bp, Homo sapiens
  source 1..357: mol_type = unassigned DNA
gaggtgcagctggtggagtctgggggaggcttggtccagcctggggggtccctgagactctcctgtgcagcctctggactcacctttagtaacttttggatgagctgggtccgccaggctccagggaaggggctggagtgggtggccaacataaagcaagatggaaatgataaatactatgtggactctgtgaagggccgattcaccatctccagagacaacgccaagaattcactgtatctgcaaatgaacagcctgagagccgaggacacggctgtgtattactgtgcgagagagtcaaactggggatttgcttttgatatctggggccaagggacaatggtcaccgtctcttca

SEQ ID NO: 471 - protein, 119 aa, Homo sapiens
EVQLVESGGGLVQPGGSLRLSCAASGLTFSNFWMSWVRQAPGKGLEWVANIKQDGNDKYYVDSVKGRFTISRDNAKNSLYLQMNSLRAEDTAVYYCARESNWGFAFDIWGQGTMVTVSS

SEQ ID NO: 472 - DNA, 327 bp, Homo sapiens; identical to SEQ ID NO: 145
  source 1..327: mol_type = unassigned DNA

SEQ ID NO: 473 - protein, 109 aa, Homo sapiens; identical to SEQ ID NO: 33

SEQ ID NO: 474 - DNA, 357 bp, Homo sapiens
  source 1..357: mol_type = unassigned DNA
gaggtgcagctggtggagtctgggggaggtttggtccagcctggggggtccctgagactctcctgtgcagcctctggactcacctttagtaacttttggatgagctgggtccgccaggctccagggaaggggctggagtgggtggccaacataaagcaagatggaagtgagaaatactatgtggactctgtgaagggccgattcaccatctccagagacaacgccaagaattcactgtatctgcaaatgaacagcctgagagccgaggacacggctgtgtattactgtgcgagagagtcaaactggggatttgcttttgatatctggggccaagggacaatggtcaccgtctcttca

SEQ ID NO: 475 - protein, 119 aa, Homo sapiens
EVQLVESGGGLVQPGGSLRLSCAASGLTFSNFWMSWVRQAPGKGLEWVANIKQDGSEKYYVDSVKGRFTISRDNAKNSLYLQMNSLRAEDTAVYYCARESNWGFAFDIWGQGTMVTVSS

SEQ ID NO: 476 - DNA, 327 bp, Homo sapiens
  source 1..327: mol_type = unassigned DNA
cagtctgtgctgactcagccaccctcagcgtctgggacccccgggcagagggtcaccatctcttgttctggaagcagctccaacatcggaagtaaaactgtaaactggtaccagcagttcccaggaacggcccccaaactcctcatctatagtaataatcggcggccctcaggggtccctgaccgattctctggctccaagtctggcacctcagcctccctggccatcagtgggctccagtctgaggatgaggctgattattactgtgcaacatgggatgacagactgaattgggtgttcggcgcagggaccaagctgaccgtccta

SEQ ID NO: 477 - protein, 109 aa, Homo sapiens
QSVLTQPPSASGTPGQRVTISCSGSSSNIGSKTVNWYQQFPGTAPKLLIYSNNRRPSGVPDRFSGSKSGTSASLAISGLQSEDEADYYCATWDDRLNWVFGAGTKLTVL

SEQ ID NO: 478 - DNA, 366 bp, Homo sapiens
  source 1..366: mol_type = unassigned DNA
caggtcaccttgaaggagtctggtcctgtgctggtgaaacccacagagaccctcacgctgacctgcaccgtctctgggttctcactcagcaatgttagaatgggtgtgagctggatccgtcagcccccagggaaggccctggagtggcttgcacacattttttcgaatgacgaaaattcctacagaacatctctgaagagcaggctcaccatctccaaggacacctccaaaagccaggtggtccttaccatgaccaacatggaccctgtggacacagccacatattactgtgcacggatagtgggagctacaacggatgatgcttttgatatctggggccaagggacaatggtcaccgtctcttca

SEQ ID NO: 479 - protein, 122 aa, Homo sapiens
QVTLKESGPVLVKPTETLTLTCTVSGFSLSNVRMGVSWIRQPPGKALEWLAHIFSNDENSYRTSLKSRLTISKDTSKSQVVLTMTNMDPVDTATYYCARIVGATTDDAFDIWGQGTMVTVSS

SEQ ID NO: 480 - DNA, 324 bp, Homo sapiens
  source 1..324: mol_type = unassigned DNA
tcctatgtgctgactcagccaccctcggtgtcagtggccccaggacagacggccaggattacctgtgggggaaacaacattggaagtaaaagtgtgcactggtaccagcagaagccaggccaggcccctgtgctggtcgtctatgatgatagcgaccggccctcagggatccctgagcgattctctggctccaactctgggaacacggccaccctgaccatcagcagggtcgaagccggggatgaggccgacttttactgtcaggtgtgggatagtagtagtgatcctgtggtattcggcggagggaccaagctgaccgtccta

SEQ ID NO: 481 - protein, 108 aa, Homo sapiens
SYVLTQPPSVSVAPGQTARITCGGNNIGSKSVHWYQQKPGQAPVLVVYDDSDRPSGIPERFSGSNSGNTATLTISRVEAGDEADFYCQVWDSSSDPVVFGGGTKLTVL

SEQ ID NO: 482 - DNA, 381 bp, Homo sapiens
  source 1..381: mol_type = unassigned DNA
gaggtgcagctggtggagtctgggggaggcttggtccagcctggggggtccctgagactctcctgtgcagcctctggattcacctttagtaactattggatgacctgggtccgccaggctccagggaaggggctggagtgggtggccagcataaagcaagatggaagtgagagatactatgtggactctgtgaagggccgattcaccatctcccgagacaccgccaagaactctctgtatctccaaatgaacagcctgcgagccgaggacacggctgtgtattactgtgcgagacctcttgtactaatggtgtatgctctacactactactactacggtatggacgtctggggccacgggaccacggtcaccgtctcctca

SEQ ID NO: 483 - protein, 127 aa, Homo sapiens
EVQLVESGGGLVQPGGSLRLSCAASGFTFSNYWMTWVRQAPGKGLEWVASIKQDGSERYYVDSVKGRFTISRDTAKNSLYLQMNSLRAEDTAVYYCARPLVLMVYALHYYYYGMDVWGHGTTVTVSS

SEQ ID NO: 484 - DNA, 336 bp, Homo sapiens
  source 1..336: mol_type = unassigned DNA
gatattgtgatgactcagtctccactctccctgcccgtcacccctggagagccggcctccatctcctgcaggtctagtcagagcctcctgcatagtaatggatacaactatttggattggtacctgcagaagccagggcagtctccacagctcctgatctatttgggttctaatcgggcctccggggtccctgacaggttcagtggcagtggatcaggcacagattttacactgaaaatcagcagagtggaggctgaggatgttggggtttattactgcatgcaagctctacaaactccgctcactttcggcggagggaccaaggtggagatcaaa

SEQ ID NO: 485 - protein, 112 aa, Homo sapiens; identical to SEQ ID NO: 461

SEQ ID NO: 486 - protein, 100 aa, Homo sapiens
QVTLKESGPVLVKPTETLTLTCTVSGFSLSNARMGVSWIRQPPGKALEWLAHIFSNDEKSYSTSLKSRLTISKDTSKSQVVLTMTNMDPVDTATYYCARI

SEQ ID NO: 487 - protein, 98 aa, Homo sapiens
EVQLVESGGGLVQPGGSLRLSCAASGFTFSSYWMSWVRQAPGKGLEWVANIKQDGSEKYYVDSVKGRFTISRDNAKNSLYLQMNSLRAEDTAVYYCAR

SEQ ID NO: 488 - protein, 98 aa, Homo sapiens
QVQLVESGGGVVQPGRSLRLSCAASGFTFSSYGMHWVRQAPGKGLEWVAVIWYDGSNKYYADSVKGRFTISRDNSKNTLYLQMNSLRAEDTAVYYCAR

SEQ ID NO: 489 - protein, 93 aa, Homo sapiens
DIVMTQSPLSLPVTPGEPASISCRSSQSLLHSNGYNYLDWYLQKPGQSPQLLIYLGSNRASGVPDRFSGSGSGTDFTLKISRVEAEDVGVYYC

SEQ ID NO: 490 - protein, 94 aa, Homo sapiens
DIVMTQSPDSLAVSLGERATINCKSSQSVLYSSNNKNYLAWYQQKPGQPPKLLIYWASTRESGVPDRFSGSGSGTDFTLTISSLQAEDVAVYYC

SEQ ID NO: 491 - protein, 89 aa, Homo sapiens
QSVLTQPPSASGTPGQRVTISCSGSSSNIGSNTVNWYQQLPGTAPKLLIYSNNQRPSGVPDRFSGSKSGTSASLAISGLQSEDEADYYC

SEQ ID NO: 492 - protein, 87 aa, Homo sapiens
SYVLTQPPSVSVAPGKTARITCGGNNIGSKSVHWYQQKPGQAPVLVIYYDSDRPSGIPERFSGSNSGNTATLTISRVEAGDEADYYC

SEQ ID NO: 493 - protein, 49 aa, Homo sapiens
QVQLVQSGAEVKKPGASVKVSCKASGYTFTGYYMHWVRQAPGQGLEWMG

SEQ ID NO: 494 - protein, 98 aa, Homo sapiens; identical to SEQ ID NO: 488

SEQ ID NO: 495 - protein, 98 aa, Homo sapiens; identical to SEQ ID NO: 488

SEQ ID NO: 496 - protein, 88 aa, Homo sapiens
DIQMTQSPSSLSASVGDRVTITCRASQGISNYLAWYQQKPGKVPKLLIYAASTLQSGVPSRFSGSGSGTDFTLTISSLQPEDVATYYC

SEQ ID NO: 497 - protein, 90 aa, Homo sapiens
QSALTQPASVSGSPGQSITISCTGTSSDVGGYNYVSWYQQHPGKAPKLMIYEVSNRPSGVSNRFSGSKSGNTASLTISGLQAEDEADYYC

SEQ ID NO: 498 - protein, 87 aa, Homo sapiens
SSELTQDPAVSVALGQTVRITCQGDSLRSYYASWYQQKPGQAPVLVIYGKNNRPSGIPDRFSGSSSGNTASLTITGAQAEDEADYYC

SEQ ID NO: 499 - protein, 13 aa, Homo sapiens
SGSSSNIGSKTVN